European Patent Specification EP 3 592 380 B1, published October 9, 2024. Title: New Universal chimeric antigen receptor T cells specific for CD22. Applicant: Cellectis SA. The sequence listing filed with the application follows.

SEQUENCE LISTING (126 sequences)

SEQ ID NO: 1 - protein, 21 aa, homo sapiens
  CD8alpha signal peptide
MALPVTALLLPLALLLHAARP

SEQ ID NO: 2 - protein, 20 aa, homo sapiens
  signal peptide
METDTLLLWVLLLWVPGSTG

SEQ ID NO: 3 - protein, 16 aa, homo sapiens
  FcgRIIIa hinge
GLAVSTISSFFPPGYQ

SEQ ID NO: 4 - protein, 45 aa, homo sapiens
  CD8alpha hinge
TTTPAPRPPTPAPTIASQPLSLRPEACRPAAGGAVHTRGLDFACD

SEQ ID NO: 5 - protein, 231 aa, homo sapiens
  IgG1 hinge
EPKSPDKTHTCPPCPAPPVAGPSVFLFPPKPKDTLMIARTPEVTCVVVDVSHEDPEVKFNWYVDGVEVHNAKTKPREEQYNSTYRVVSVLTVLHQDWLNGKEYKCKVSNKALPAPIEKTISKAKGQPREPQVYTLPPSRDELTKNQVSLTCLVKGFYPSDIAVEWESNGQPENNYKTTPPVLDSDGSFFLYSKLTVDKSRWQQGNVFSCSVMHEALHNHYTQKSLSLSPGK

SEQ ID NO: 6 - protein, 24 aa, homo sapiens
  CD8alpha transmembrane domain
IYIWAPLAGTCGVLLLSLVITLYC

SEQ ID NO: 7 - protein, 27 aa, homo sapiens
  41BB transmembrane domain
IISFFLALTSTALLFLLFFLTLRFSVV

SEQ ID NO: 8 - protein, 42 aa, homo sapiens
  Fragment of 4-1BB (residues 214-255)
KRGRKKLLYIFKQPFMRPVQTTQEEDGCSCRFPEEEEGGCEL

SEQ ID NO: 9 - protein, 112 aa, homo sapiens
  fragment of T-cell surface glycoprotein CD3 zeta chain
RVKFSRSADAPAYQQGQNQLYNELNLGRREEYDVLDKRRGRDPEMGGKPRRKNPQEGLYNELQKDKMAEAYSEIGMKGERRRGKGHDGLYQGLSTATKDTYDALHMQALPPR

SEQ ID NO: 10 - protein, 15 aa, artificial sequence
  G4Sx3 linker sequence
GGGGSGGGGSGGGGS

SEQ ID NO: 11 - protein, 117 aa, artificial sequence
  972- heavy chain
EVQLVQSGGGVVRPGGSLRLPCAASGFTFDDYGMSWVRQAPGKGLEWVSGINWNGGSTGYADSVKGRFTISRDNAKNSLYLQMNSLRAEDTALYHCARGGDDAFDIWGQGTMVTVSS

SEQ ID NO: 12 - protein, 108 aa, artificial sequence
  972- light chain variable region
RIVMTQSPGTLSVSPGETATLSCRASQSFSNMLAWYQQKSGQPPRLLIYGVSTRAAGVPARFSGSGSGTEFTLTISNLQSEDFAVYYCQQYGDWPRYTFGQGTKVERK

SEQ ID NO: 13 - protein, 124 aa, artificial sequence
  971- heavy chain
QVQLQQSGPGLVKPSQTLSLTCAISGDSVSSNSAAWNWIRQSPSRGLEWLGRTYYRSKWYNDYAVSVKSRITINPDTSKNQFSLQLNSVTPEDTAVYYCAREVTGDLEDAFDIWGQGTMVTVSS

SEQ ID NO: 14 - protein, 107 aa, artificial sequence
  971- light chain
DIQMTQSPSSLSASVGDRVTITCRASQTIWSYLNWYQQRPGKAPNLLIYAASSLQSGVPSRFSGRGSGTDFTLTISSLQAEDFATYYCQQSYSIPQTFGQGTKLEIK

SEQ ID NO: 15 - protein, 461 aa, artificial sequence
  972-v1 polypolypeptide CAR sequence
EVQVLESGGGLVQPGGSLRLSCAASGFTFSSYAMSWVRQAPGKGLEWVSAISGSGGSTNYADSVKGRFTISRDNSKNTLYLQMNSLRAEDTAVYYCAGSSGWSEYWGQGTLVTVSSGGGGSGGGGSGGGGSDIQMTQSPSSLSASVGDRVTITCRASQGIRNNLAWYQQKPGKAPKRLIYAASNLQSGVPSRFTGSGSGTEFTLIVSSLQPEDFATYYCLQHHSYPLTSGGGTKVEIKTTTPAPRPPTPAPTIASQPLSLRPEACRPAAGGAVHTRGLDFACDIYIWAPLAGTCGVLLLSLVITLYCKRGRKKLLYIFKQPFMRPVQTTQEEDGCSCRFPEEEEGGCELRVKFSRSADAPAYQQGQNQLYNELNLGRREEYDVLDKRRGRDPEMGGKPRRKNPQEGLYNELQKDKMAEAYSEIGMKGERRRGKGHDGLYQGLSTATKDTYDALHMQALPPR

SEQ ID NO: 16 - protein, 647 aa, artificial sequence
  972-v3 polypolypeptide CAR sequence
EVQVLESGGGLVQPGGSLRLSCAASGFTFSSYAMSWVRQAPGKGLEWVSAISGSGGSTNYADSVKGRFTISRDNSKNTLYLQMNSLRAEDTAVYYCAGSSGWSEYWGQGTLVTVSSGGGGSGGGGSGGGGSDIQMTQSPSSLSASVGDRVTITCRASQGIRNNLAWYQQKPGKAPKRLIYAASNLQSGVPSRFTGSGSGTEFTLIVSSLQPEDFATYYCLQHHSYPLTSGGGTKVEIKEPKSPDKTHTCPPCPAPPVAGPSVFLFPPKPKDTLMIARTPEVTCVVVDVSHEDPEVKFNWYVDGVEVHNAKTKPREEQYNSTYRVVSVLTVLHQDWLNGKEYKCKVSNKALPAPIEKTISKAKGQPREPQVYTLPPSRDELTKNQVSLTCLVKGFYPSDIAVEWESNGQPENNYKTTPPVLDSDGSFFLYSKLTVDKSRWQQGNVFSCSVMHEALHNHYTQKSLSLSPGKIYIWAPLAGTCGVLLLSLVITLYCKRGRKKLLYIFKQPFMRPVQTTQEEDGCSCRFPEEEEGGCELRVKFSRSADAPAYQQGQNQLYNELNLGRREEYDVLDKRRGRDPEMGGKPRRKNPQEGLYNELQKDKMAEAYSEIGMKGERRRGKGHDGLYQGLSTATKDTYDALHMQALPPR

SEQ ID NO: 17 - protein, 464 aa, artificial sequence
  971-v1 polypolypeptide CAR sequence
QVQLQQSGGGLVKPGASLKLSCVTSGFTFRKFGMSWVRQTSDKRLEWVASISTGGYNTYYSDNVKGRFTISRENAKNTLYLQMSSLKSEDTALYYCTRGYSSTSYAMDYWGQGTTVTVGGGGSGGGGSGGGGSDIELTQSPASLSVATGEKVTIRCMTSTDIDDDMNWYQQKPGEPPKFLISEGNTLRPGVPSRFSSSGTGTDFVFTIENTLSEDVGDYYCLQSFNVPLTFGDGTKLEKALTTTPAPRPPTPAPTIASQPLSLRPEACRPAAGGAVHTRGLDFACDIYIWAPLAGTCGVLLLSLVITLYCKRGRKKLLYIFKQPFMRPVQTTQEEDGCSCRFPEEEEGGCELRVKFSRSADAPAYQQGQNQLYNELNLGRREEYDVLDKRRGRDPEMGGKPRRKNPQEGLYNELQKDKMAEAYSEIGMKGERRRGKGHDGLYQGLSTATKDTYDALHMQALPPR

SEQ ID NO: 18 - protein, 650 aa, artificial sequence
  971-v3 polypolypeptide CAR sequence
QVQLQQSGGGLVKPGASLKLSCVTSGFTFRKFGMSWVRQTSDKRLEWVASISTGGYNTYYSDNVKGRFTISRENAKNTLYLQMSSLKSEDTALYYCTRGYSSTSYAMDYWGQGTTVTVGGGGSGGGGSGGGGSDIELTQSPASLSVATGEKVTIRCMTSTDIDDDMNWYQQKPGEPPKFLISEGNTLRPGVPSRFSSSGTGTDFVFTIENTLSEDVGDYYCLQSFNVPLTFGDGTKLEKALEPKSPDKTHTCPPCPAPPVAGPSVFLFPPKPKDTLMIARTPEVTCVVVDVSHEDPEVKFNWYVDGVEVHNAKTKPREEQYNSTYRVVSVLTVLHQDWLNGKEYKCKVSNKALPAPIEKTISKAKGQPREPQVYTLPPSRDELTKNQVSLTCLVKGFYPSDIAVEWESNGQPENNYKTTPPVLDSDGSFFLYSKLTVDKSRWQQGNVFSCSVMHEALHNHYTQKSLSLSPGKIYIWAPLAGTCGVLLLSLVITLYCKRGRKKLLYIFKQPFMRPVQTTQEEDGCSCRFPEEEEGGCELRVKFSRSADAPAYQQGQNQLYNELNLGRREEYDVLDKRRGRDPEMGGKPRRKNPQEGLYNELQKDKMAEAYSEIGMKGERRRGKGHDGLYQGLSTATKDTYDALHMQALPPR

SEQ ID NO: 19 - protein, 530 aa, artificial sequence
  TAL binding domain  TRAC_T01-L
LTPQQVVAIASNGGGKQALETVQRLLPVLCQAHGLTPQQVVAIASNNGGKQALETVQRLLPVLCQAHGLTPQQVVAIASNGGGKQALETVQRLLPVLCQAHGLTPEQVVAIASHDGGKQALETVQRLLPVLCQAHGLTPEQVVAIASHDGGKQALETVQRLLPVLCQAHGLTPEQVVAIASHDGGKQALETVQRLLPVLCQAHGLTPEQVVAIASNIGGKQALETVQALLPVLCQAHGLTPEQVVAIASHDGGKQALETVQRLLPVLCQAHGLTPEQVVAIASNIGGKQALETVQALLPVLCQAHGLTPQQVVAIASNNGGKQALETVQRLLPVLCQAHGLTPEQVVAIASNIGGKQALETVQALLPVLCQAHGLTPQQVVAIASNGGGKQALETVQRLLPVLCQAHGLTPEQVVAIASNIGGKQALETVQALLPVLCQAHGLTPQQVVAIASNGGGKQALETVQRLLPVLCQAHGLTPEQVVAIASHDGGKQALETVQRLLPVLCQAHGLTPQQVVAIASNGGGRPALE

SEQ ID NO: 20 - protein, 530 aa, artificial sequence
  TAL binding domain TRAC_T01-R
LTPEQVVAIASHDGGKQALETVQRLLPVLCQAHGLTPQQVVAIASNGGGKQALETVQRLLPVLCQAHGLTPEQVVAIASHDGGKQALETVQRLLPVLCQAHGLTPEQVVAIASNIGGKQALETVQALLPVLCQAHGLTPQQVVAIASNNGGKQALETVQRLLPVLCQAHGLTPEQVVAIASHDGGKQALETVQRLLPVLCQAHGLTPQQVVAIASNGGGKQALETVQRLLPVLCQAHGLTPQQVVAIASNNGGKQALETVQRLLPVLCQAHGLTPQQVVAIASNNGGKQALETVQRLLPVLCQAHGLTPQQVVAIASNGGGKQALETVQRLLPVLCQAHGLTPEQVVAIASNIGGKQALETVQALLPVLCQAHGLTPEQVVAIASHDGGKQALETVQRLLPVLCQAHGLTPEQVVAIASNIGGKQALETVQALLPVLCQAHGLTPEQVVAIASHDGGKQALETVQRLLPVLCQAHGLTPQQVVAIASNNGGKQALETVQRLLPVLCQAHGLTPQQVVAIASNGGGRPALE

SEQ ID NO: 21 - DNA, 1464 bp, artificial
  CAR 1
atggctctgcccgtcaccgctctgctgctgccactggccctgctgctgcacgcagccagaccccaggtgcagctgcagcagagcggccctggcctggtgaagccatctcagacactgagcctgacctgcgccatctctggcgacagcgtgagctccaactctgccgcctggaattggatcagacagtccccatctaggggcctggagtggctgggacgcacatactatcggtccacctggtacaacgactatgccgtgtccgtgaagtctcgcatcacaatcaaccccgatacctctaagaatcagttcagcctgcagctgaattccgtgacacctgaggacaccgccgtgtactattgcgccagagaggtgagcggcacatccgcctttgatatctggggccagggcacaatggtgaccgtgtctggaggaggaggaagcggaggaggaggatccggcggcggcggctctgacatccagatgacccagagcccttctagcctgagcgcctccgtgggcgatcgcgtgacaatcacctgtcgggcctctcagagcatctcctcttacctgaactggtatcagcagaagcccggcaaggcccctaagctgctgatctacgcagcaagctccctgcagtccggagtgccatctcggttctccggctctggcagcggcacagactttacactgaccatctctagcctgcagcctgaggatttcgccacctactattgccagcagtcctattctacaccactgacctttggcggcggcaccaagctggagatcaagaccacaaccccagcacccagaccccctacacctgcaccaaccatcgcaagccagccactgtccctgcgccctgaggcatgtaggccagcagcaggaggagcagtgcacaccaggggcctggacttcgcctgcgatatttacatctgggcaccactggcaggaacatgtggcgtgctgctcctgagcctggtcatcaccctgtactgcaagagaggcaggaagaagctgctgtatatcttcaagcagcccttcatgcggcccgtgcagacaacccaggaggaggacggctgctcctgtaggttcccagaagaggaggagggcggctgtgagctgagagtgaagtttagcaggtccgccgatgcaccagcataccagcagggacagaatcagctgtataacgagctgaatctgggccggagagaggagtacgacgtgctggataagaggaggggaagggatcctgagatgggaggcaagccccggagaaagaaccctcaggagggcctgtacaatgagctgcagaaggacaagatggccgaggcctatagcgagatcggcatgaagggagagaggcgccggggcaagggacacgatggcctgtaccagggcctgtccacagccaccaaggacacctatgatgccctgcatatgcaggcactgcctccaaggtga

SEQ ID NO: 22 - DNA, 1479 bp, artificial sequence
  CAR 2
atggctctgcccgtcaccgctctgctgctgccactggccctgctgctgcacgcagccagaccccaggtgcagctgcagcagagcggccctggcctggtgaagccatcccagaccctgtctctgacatgcgccatcagcggcgactccgtgagctccaactctgccgcctggaattggatcagacagtccccatctaggggcctggagtggctgggaaggacctactatcggtccaagtggtacaacgactatgccgtgtctgtgaagagccgcatcaccatcaaccccgatacatccaagaatcagttctctctgcagctgaatagcgtgacccctgaggacacagccgtgtactattgcgccagagcctctatgaccggcggctacagctatggcgacgcctttgatatctggggccagggcacactggtgaccgtgtccggcggcggcggctctggaggaggaggaagcggaggaggaggatccgccatccgcatgacacagagcccttctagcctgagcgcctccgtgggcgatcgcgtgacaatcacctgtcgggcctctcagagcatctcctcttacctgaactggtatcagcagaagcccggcaaggcccctaagctgctgatctacgcagcaagctccctgcagagcggagtgccatcccggttctccggatctggaagcggaaccgacttttccctgacaatctctagcctgcagcctgaggattccgccacctactattgccagcagacatattctaccccactgacattcggccagggcacaaaggtggagatcaagaccacaaccccagcacccagaccccctacccctgcaccaacaatcgcctctcagcccctgagcctgcgccctgaggcatgtaggccagcagcaggaggagcagtgcacaccaggggcctggactttgcctgcgatatttacatctgggcaccactggcaggaacctgtggcgtgctgctcctgagcctggtcatcaccctgtactgcaagagaggcaggaagaagctgctgtatatcttcaagcagcccttcatgcggcccgtgcagacaacccaggaggaggacggctgctcctgtaggttcccagaagaggaggagggcggctgtgagctgagagtgaagttttccaggtctgccgatgcaccagcataccagcagggacagaatcagctgtataacgagctgaatctgggccggagagaggagtacgacgtgctggataagaggaggggacgggatcctgagatgggaggcaagccccggagaaagaaccctcaggagggcctgtacaatgagctgcagaaggacaagatggccgaggcctatagcgagatcggcatgaagggagagaggcgccggggcaagggacacgatggcctgtaccagggcctgtccacagccaccaaggacacctatgatgccctgcatatgcaggcactgcctccaaggtga

SEQ ID NO: 23 - DNA, 1467 bp, artificial sequence
  CAR 3
atggctctgcccgtcaccgctctgctgctgccactggccctgctgctgcacgcagccagaccccaggtgcagctgcagcagagcggccctggcctggtggagccaagccagacactgtccctgacctgcgccatctctggcgacagcgtgagctccgattccgtggcctggaactggatcaggcagtctccaagccggggcctggagtggctgggcagaacatactataggtctacctggtacaatgactatgccggctccgtgaagtctcgcatcacaatcaaccccgataccagcaagaatcagttctccctgcagctgacatctgtgacccctgaggacacagccgtgtactattgcaccagatccaggcacaacacatttcggggaatggacgtgtggggacagggaaccacagtgaccgtgagcggaggaggaggatccggcggaggaggctctggaggaggaggaagcgacatcgtgatgacccagagcccttctagcctgtccgcctctgtgggcgatagagtgacaatcacctgtagggcctcccagaccatctcctcttacctgaactggtatcagcagaagcccggcaaggcccctaagctgctgatctacgacgcaagctccctgcagtctggagtgccaagcagattcagcggctccggctctggcaccgactttacactgaccatcaattccctgcagcctgaggatttcgccacatactattgccagcagtcttataccacaccaatcacatttggccagggcacccgcctggagatcaagaccacaaccccagcacccagaccccctacacctgcaccaaccatcgcatcccagccactgtctctgcggcccgaggcatgtaggccagcagcaggaggagcagtgcacaccaggggcctggacttcgcctgcgatatttacatctgggcaccactggcaggaacctgtggcgtgctgctcctgagcctggtcatcaccctgtactgcaagcgcggccggaagaagctgctgtatatcttcaagcagcccttcatgcggcccgtgcagacaacccaggaggaggacggctgctcctgtaggttcccagaagaggaggagggaggatgtgagctgagggtgaagtttagccggtccgccgatgcaccagcataccagcagggccagaatcagctgtataacgagctgaatctgggccggagagaggagtacgacgtgctggataagaggaggggaagggatcctgagatgggaggcaagccccggagaaagaaccctcaggagggcctgtacaatgagctgcagaaggacaagatggccgaggcctattctgagatcggcatgaagggagagaggcgccggggcaagggacacgatggcctgtaccagggcctgagcacagccaccaaggacacctatgatgccctgcatatgcaggcactgcctccaaggtga

SEQ ID NO: 24 - DNA, 1467 bp, artificial sequence
  CAR 4
atggctctgcccgtcaccgctctgctgctgccactggccctgctgctgcacgcagccagaccccaggtgcagctgcagcagagcggccctggcctggtggagccaagccagacactgtccctgacctgcgccatctctggcgacagcgtgagctccaacagcgccgcatggaattggatcaggcagtccccatctcggggcctggagtggctgggcagaacatactataggtccacctggtacaacgactatgccggctccgtgaagtctcgcatcacaatcaaccccgataccagcaagaatcagttctccctgcagctgacatctgtgacccctgaggacacagccgtgtactattgcaccagaagcaggcacaatacatttcggggaatggacgtgtggggacagggcacactggtgaccgtgagcggaggaggaggatccggcggaggaggctctggcggcggcggcagcgacatccagctgacccagtccccttctagcctgagcgcctccgtgggcgatagagtgacaatcacctgtagggcctctcagagcatctcctcttacctgaactggtatcagcagaagcccggcaaggcccctaagctgctgatctacgcagcaagctccctgcagtctggagtgccaagcagattctccggctctggcagcggcaccgactttacactgaccatctctagcctgcagcctgaggatttcgccacatactattgccagcagtcctattctacaccactgacctttggcggcggcaccaaggtggagatcaagaccacaaccccagcacccagaccccctacacctgcaccaaccatcgcatcccagccactgtctctgcggcccgaggcatgtaggccagcagcaggaggagcagtgcacaccaggggcctggacttcgcctgcgatatctacatttgggcaccactggcaggaacctgtggcgtgctgctcctgagcctggtcatcaccctgtactgcaagcgcggccggaagaagctgctgtatatcttcaagcagcccttcatgcggcccgtgcagacaacccaggaggaggacggctgctcctgtcggttcccagaagaggaggagggaggatgtgagctgagggtgaagtttagccggtccgccgatgcaccagcataccagcagggccagaatcagctgtataacgagctgaatctgggccggagagaggagtacgacgtgctggataagaggaggggaagggatcctgagatgggaggcaagccccggagaaagaaccctcaggagggcctgtacaatgagctgcagaaggacaagatggccgaggcctattccgagatcggcatgaagggagagaggcgccggggcaagggacacgatggcctgtaccagggcctgtctacagccaccaaggacacctatgatgccctgcatatgcaggcactgcctccaaggtga

SEQ ID NO: 25 - DNA, 1455 bp, artificial sequence
  CAR 5 7
atggctctgcccgtcaccgctctgctgctgccactggccctgctgctgcacgcagccagaccccaggtgcagctgcagcagagcggccctggcctggtggagccaagccagaccctgtccctgacatgcgccatctctggcgacagcgtgagctccgattctgtggcctggaactggatcaggcagagcccaagccggggcctggagtggctgggcagaacctactataggtccacatggtacaatgactatgccggctccgtgaagtctcggatcaccatcaaccccgatacatccaagaatcagttctctctgcagctgaacagcgtgacccctgaggacacagccgtgtactattgcgccagagacaggaatggcatggacgtgtggggccagggaaccatggtgacagtgtccggaggaggcggctctggaggaggaggaagcggaggaggaggatccgacatcgtgatgacccagagcccttctagcctgtctgccagcgtgggcgatagagtgacaatcacctgtagggcctcccagtctatctcctcttacctgaactggtatcagcagaagcccggcaaggcccctaagctgctgatctacgatgcctctaatctggagacaggcgtgccaagcagattcagcggctccggctctggcacagacttcaccttcaccatcacatccctgcagcctgaggatttcgccacctactattgccagcagtcttataccacaccactgacctttggcggcggcacaaaggtggagatcaagaccacaaccccagcacccagaccccctacccctgcaccaacaatcgcctctcagcccctgagcctgcggcccgaggcctgtaggccagcagcaggaggagcagtgcacaccaggggcctggactttgcctgcgatatttacatctgggcaccactggcaggaacctgtggcgtgctgctcctgagcctggtcatcaccctgtactgcaagcgcggccggaagaagctgctgtatatcttcaagcagcccttcatgcggcccgtgcagacaacccaggaggaggacggctgctcctgtcggttcccagaagaggaggagggaggatgtgagctgagggtgaagtttagccggtccgccgatgcaccagcataccagcagggacagaaccagctgtataacgagctgaatctgggccggagagaggagtacgacgtgctggataagaggaggggacgggaccctgagatgggaggcaagccccggagaaagaaccctcaggagggcctgtacaatgagctgcagaaggacaagatggccgaggcctatagcgagatcggcatgaagggagagaggcgccggggcaagggacacgatggcctgtaccagggcctgtccaccgccacaaaggacacctatgatgccctgcatatgcaggcactgcctccaaggtga

SEQ ID NO: 26 - DNA, 1464 bp, artificial sequence
  CAR 6-8
atggctctgcccgtcaccgctctgctgctgccactggccctgctgctgcacgcagcccgccctcaggtgcagctgcagcagtccggcccaggcctggtgaagccatcccagacactgtctctgacctgcgccatcagcggcgactccgtgagctcctctagcgccgcctggaactggatcagacagtctcctagcaggggcctggagtggctgggaaggacctactatcggtccgcctggtacaatgactatgccgtgtctgtgaagagcagaatcacaatcaaccccgatacctccaagaatcagttctctctgcagctgaacagcgtgacacctgaggataccgccgtgtactattgcgccagagagagcgtgctgctggacggaatggacgtgtggggaaggggaaccacagtgacagtgtccggaggaggcggctctggaggaggaggaagcggaggaggaggatccgccatcaggatgacacagtccccatctaccctgagcgcctccgtgggcgaccgcgtgacaatcacctgtcgggcctctcagagcatctccacctacctgaattggtatcagcagaaggccggcaaggccccaagactgctgatccacgatgcatcctctctgcagagcggagtgccatccaggttctctggaagcggatccggcacagactttacactgaccatcagctccctgcagcctgaggatttcgccacctactattgccagcagtcttacagcacaccactgacctttggcggcggcacaaaggtggagatcaagaccacaaccccagcacccagaccccctacacctgcaccaaccatcgcctctcagcctctgagcctgcgcccagaggcatgtaggccagcagcaggaggagcagtgcacaccagaggcctggactttgcctgcgatatttatatctgggcacctctggcaggaacatgtggcgtgctgctcctgagcctggtcatcaccctgtactgcaagagaggcaggaagaagctgctgtatatcttcaagcagccctttatgcgccctgtgcagacaacccaggaggaggacggctgcagctgtcggttcccagaagaggaggagggcggctgtgagctgagagtgaagttttccaggtctgccgatgcaccagcataccagcagggacagaaccagctgtataacgagctgaatctgggccggagagaggagtacgacgtgctggataagaggaggggaagggaccccgagatgggaggcaagcctcggagaaagaacccacaggagggcctgtacaatgagctgcagaaggacaagatggccgaggcctattctgagatcggcatgaagggagagaggcgccggggcaagggacacgatggcctgtaccagggcctgagcacagccaccaaggacacctatgatgccctgcatatgcaggcactgcctccaaggtga

SEQ ID NO: 27 - DNA, 1485 bp, artificial sequence
  CAR 7 -9
atggctctgcccgtcaccgctctgctgctgccactggccctgctgctgcacgcagccagaccccaggtgcagctgcagcagagcggccctggcctggtgcagccatcccagacactgtctctgacctgcgtgatcagcggcgactccgtgagctccaactctgccacatggaattggatcagacagagcccatccaggggcctggagtggctgggacgcacctactatcggagcaagtggtacaacgactatgccgtgtctgtgaagagcagaatcacaatcaaccccgatacctctaagaatcagttcagcctgcagctgaattccgtgacacctgaggataccgccgtgtactattgcgccagggacggcgatggaggaagctactatgactactattactatggcatggacgtgtggggccagggcaccacagtgacagtgtctggaggaggaggaagcggaggaggaggatccggcggcggcggctctgacatccagctgacacagtccccttctagcctgtctaccagcgtgggcgatcgcgtgacaatcacctgtcgggcctcccagtctatcagcacctacctgaactggtatcagcagaagcccggcaaggcccctaagctgctgatctacgcagcaagcaatctgcagtccggagtgccatctcgcttctccggctctggcagcggcacagactttacactgaccatctcctctctgcagcctgaggatttcgccacctacttttgccagcagtcctataccacaccaatcacattcggccagggcaccagactggagatcaagaccacaaccccagcacccaggccccctacacctgcaccaaccatcgcaagccagccactgtccctgcgccctgaggcatgtaggccagcagcaggaggagcagtgcacaccagaggcctggactttgcctgcgatatttacatctgggcaccactggcaggaacatgtggcgtgctgctcctgagcctggtcatcaccctgtactgcaagagaggcaggaagaagctgctgtatatcttcaagcagcccttcatgcggcccgtgcagacaacccaggaggaggacggctgctcttgtcggttcccagaagaggaggagggcggctgtgagctgagagtgaagttttccaggtctgccgatgcaccagcataccagcagggacagaaccagctgtataacgagctgaatctgggccggagagaggagtacgacgtgctggataagaggaggggacgggaccctgagatgggaggcaagccccggagaaagaaccctcaggagggcctgtacaatgagctgcagaaggacaagatggccgaggcctatagcgagatcggcatgaagggagagaggcgccggggcaagggacacgatggcctgtaccagggcctgtccacagccaccaaggacacctatgatgccctgcatatgcaggcactgcctccaaggtga

SEQ ID NO: 28 - DNA, 1455 bp, artificial sequence
  CAR 8 12
atggctctgcccgtcaccgctctgctgctgccactggccctgctgctgcacgcagccagaccccaggtgcagctgcagcagtccggccctggcctggtgaagccatctcagacactgagcctgacctgcgccatctccggcgactctgtgagctccaactccgccgcctggaattggatcagacagagcccatccaggggcctggagtggctgggacgcacctactatcggagcgcctggtacaacgactatgccgtgagcgtgaagtccagaatcacaatcaaccccgatacctctaagaatcagttcagcctgcagctgtctagcgtgacacctgaggataccgccgtgtactattgcgccagggacgtggagggctttgattactggggccagggcacactggtgaccgtgtccggcggcggcggctctggaggaggaggaagcggaggaggaggatccgacatcgtgatgacacagaccccttcctctctgtctgccagcgtgggcgatcgcgtgacaatcacctgtcgggcctcccagtctatcagctcctacctgaattggtatcagcagaagcccggcaaggcccctaagctgctgatctacgcagcatctagcctgcagtccggagtgccatctcgcttcagcggatccggctctggcacagactttacactgaccatctcctctctgcagcctgaggatttcgccacctactattgccagcagagctattccacaccaatcacctttggccagggcacaagactggagatcaagaccacaaccccagcacccaggccccctacacctgcaccaaccatcgcaagccagccactgtccctgcgccctgaggcatgtaggccagcagcaggaggagcagtgcacaccagaggcctggacttcgcctgcgatatttacatctgggcaccactggcaggaacatgtggcgtgctgctcctgagcctggtcatcaccctgtactgcaagagaggcaggaagaagctgctgtatatcttcaagcagcccttcatgcggcccgtgcagacaacccaggaggaggacggctgcagctgtcggttcccagaagaggaggagggcggctgtgagctgagagtgaagttttctaggagcgccgatgcaccagcataccagcagggacagaaccagctgtataacgagctgaatctgggccggagagaggagtacgacgtgctggataagaggaggggacgggaccctgagatgggaggcaagccccggagaaagaaccctcaggagggcctgtacaatgagctgcagaaggacaagatggccgaggcctattctgagatcggcatgaagggagagaggcgccggggcaagggacacgatggcctgtaccagggcctgagcacagccaccaaggacacctatgatgccctgcatatgcaggcactgcctccaaggtga

SEQ ID NO: 29 - DNA, 1470 bp, artificial sequence
  CAR 9 13
atggctctgcccgtcaccgctctgctgctgcctctggccctgctgctgcacgcagcccgcccacaggtgcagctgcagcagagcggccccggcctggtgaagcctagccagacactgtccctgacctgcgcaatctccggcgacagcgtgtccggaaacagggccacatggaattggatcagacagtctccaagcaggggcctggagtggctgggaaggacctactatcggtccgcctggtacaacgactatgccgtgtctgtgaagggccgcatcacattcaacccagataccagcaagaatcagttttccctgcagctgaattctgtgacacccgaggataccgccgtgtactattgcgccagaggcgagagcggagcagcagcagacgccttcgatatctggggccagggcaccacagtgacagtgagcggaggaggaggatccggcggaggaggctctggcggcggcggcagcgacatccagctgacccagagcccaccttccctgtctgccagcgtgggcgatcgcgtgacaatcacctgtcgggcctcccagtctatcagctcctacctgaactggtatcagcagaagccaggcaaggcccccaagctgctgatctacgcagcatctagcctgcagtctggagtgccaagcagattcagcggatccggattcggcacagactttacactgaccatctcctctctgcagcccgaggatttcgccacctactattgccagcagtcttatagcacacctcagacctttggccagggcaccaaggtggacatcaagaccacaacccctgcaccaagaccaccaacaccagcacctaccatcgcatcccagccactgtctctgcgccccgaggcatgtaggcctgcagcaggcggcgccgtgcacaccaggggcctggactttgcctgcgatatttacatctgggcacctctggcaggaacatgtggcgtgctgctcctgagcctggtcatcaccctgtactgcaagagaggcaggaagaagctgctgtatatcttcaagcagcccttcatgcggcccgtgcagacaacccaggaggaggacggctgctcctgtaggttccctgaagaggaggagggcggctgtgagctgagagtgaagttttccaggtctgccgatgcaccagcataccagcagggacagaatcagctgtataacgagctgaatctgggccggagagaggagtacgacgtgctggataagaggaggggacgggatcccgagatgggaggcaagccacggagaaagaacccccaggagggcctgtacaatgagctgcagaaggacaagatggccgaggcctattctgagatcggcatgaagggagagaggcgccggggcaagggacacgatggcctgtaccagggcctgtccacagccaccaaggacacctatgatgccctgcatatgcaggcactgcctccaaggtga

SEQ ID NO: 30 - DNA, 1470 bp, artificial sequence
  CAR 10 15
atggctctgcccgtcaccgctctgctgctgccactggccctgctgctgcacgcagccagaccccaggtgcagctggtgcagagcggagcagaggtgaagaagcctggcgccagcgtgaaggtgtcctgcaaggcctctggctacacattcaccagctactatatgcactgggtgcggcaggcccctggccagggcctggagtggatgggcatcatcaacccatccggcggctccacctcttacgcccagaagtttcagggcagagtgacaatgaccagggacacaagcacctccacagtgtatatggagctgagctccctgagatccgaggatacagccgtgtactattgcgccagggaggactctggaagcggagccttcgatatctggggccagggcaccctggtgacagtgtctggaggaggaggaagcggaggaggaggatccggcggcggcggctctgagatcgtgctgacccagtctccactgagcctgccagtgacacctggcgagccagcctccatctcttgtcgctctagccggtccctgctgtcttaccacggctacaattatctggactggtatctgcagaagccaggccagagcccccagctgctgatcttcgtgggatccaacagggcccctggcgtgcctgaccggttcagcggatccggatctggaaccgacttcaccctgaacatctctagagtggaggccgaggatgtgggcgtgtactattgcatgcagagcctgcagaccccaagaacatttggccagggcaccaaggtggagatcaagaccacaaccccagcacccaggccccctacccctgcaccaacaatcgcaagccagccactgtccctgcgccctgaggcatgtaggccagcagcaggaggagcagtgcacaccaggggcctggactttgcctgcgatatctacatttgggcaccactggcaggaacctgtggcgtgctgctcctgagcctggtcatcaccctgtactgcaagagaggcaggaagaagctgctgtatatcttcaagcagccttttatgcgcccagtgcagacaacccaggaggaggacggctgctcctgtaggttcccagaagaggaggagggaggatgtgagctgagagtgaagtttagcaggtccgccgatgcacctgcataccagcagggacagaaccagctgtataacgagctgaatctgggccggagagaggagtacgacgtgctggataagaggaggggacgggaccccgagatgggaggcaagccccggagaaagaaccctcaggagggcctgtacaatgagctgcagaaggacaagatggccgaggcctattccgagatcggcatgaagggagagaggcgccggggcaagggacacgatggcctgtaccagggcctgtctaccgccacaaaggacacctatgatgccctgcatatgcaggcactgcctccaaggtga

SEQ ID NO: 31 - DNA, 1473 bp, artificial sequence
  CAR 11 prox 16 m971
atggctctgcccgtcaccgctctgctgctgccactggccctgctgctgcacgcagcaagaccacaggtgcagctgcagcagagcggccctggcctggtgaagccaagccagacactgtccctgacctgcgccatcagcggcgattccgtgagctccaactccgccgcctggaattggatcaggcagtccccttctcggggcctggagtggctgggaaggacatactatcggtctaagtggtacaacgattatgccgtgtctgtgaagagcagaatcacaatcaaccctgacacctccaagaatcagttctctctgcagctgaatagcgtgacaccagaggacaccgccgtgtactattgcgccagggaggtgaccggcgacctggaggatgcctttgacatctggggccagggcacaatggtgaccgtgtctagcggaggaggaggatccggaggaggaggatctggcggcggcggcagcgatatccagatgacacagtccccatcctctctgagcgcctccgtgggcgacagagtgacaatcacctgtagggcctcccagaccatctggtcttacctgaactggtatcagcagaggcccggcaaggcccctaatctgctgatctacgcagcaagctccctgcagagcggagtgccatccagattctctggcaggggctccggcacagacttcaccctgaccatctctagcctgcaggccgaggacttcgccacctactattgccagcagtcttatagcatcccccagacatttggccagggcaccaagctggagatcaagaccacaaccccagcaccaaggccacctacacctgcaccaaccatcgcctctcagcccctgagcctgagacctgaggcatgtaggccagcagcaggaggagcagtccatacaaggggtctggattttgcatgcgacatctacatctgggcacctctggcaggaacatgtggcgtgctcctgctcagcctggtcatcaccctgtactgcaagagaggcaggaagaagctgctgtatatcttcaagcagcccttcatgcgccccgtgcagacaacccaggaggaggatggctgctcctgtaggttcccagaagaggaggagggaggatgtgagctgcgcgtgaagttttcccggtctgccgacgcacctgcataccagcagggccagaaccagctgtataacgagctgaatctgggccggagagaggagtacgatgtgctggacaagaggcgcggcagagatccagagatgggcggcaagccccggagaaagaaccctcaggagggcctgtacaatgagctgcagaaggataagatggccgaggcctattctgagatcggcatgaagggagagaggcgccggggcaagggacacgacggactgtaccagggactgagcacagccaccaaggatacctatgacgccctgcatatgcaggcactgcctccaaggtga

SEQ ID NO: 32 - DNA, 1704 bp, artificial sequence
  1 QR3
atggctctgcccgtcaccgctctgctgctgccactggccctgctgctgcacgccgccagacccggcggaggaggctcttgcccctacagcaaccccagcctgtgctctggcggcggcggcagcggaggcggcggctcccaggtgcagctgcagcagagcggccctggcctggtgaagccatctcagacactgagcctgacctgcgccatctctggcgacagcgtgagctccaactctgccgcctggaattggatcagacagtccccatctaggggcctggagtggctgggacgcacatactatcggtccacctggtacaacgactatgccgtgtccgtgaagtctcgcatcacaatcaaccccgatacctctaagaatcagttcagcctgcagctgaattccgtgacacctgaggacaccgccgtgtactattgcgccagagaggtgagcggcacatccgcctttgatatctggggccagggcacaatggtgaccgtgtctggaggaggaggaagcggaggaggaggatccggcggcggcggctctgacatccagatgacccagagcccttctagcctgagcgcctccgtgggcgatcgcgtgacaatcacctgtcgggcctctcagagcatctcctcttacctgaactggtatcagcagaagcccggcaaggcccctaagctgctgatctacgcagcaagctccctgcagtccggagtgccatctcggttctccggctctggcagcggcacagactttacactgaccatctctagcctgcagcctgaggatttcgccacctactattgccagcagtcctattctacaccactgacctttggcggcggcaccaagctggagatcaagggaagtggaggaggaggaagttgtccctattcaaacccatccctgtgcagcggaggaggaggaagcgaactgcctactcagggaacattcagcaacgtgtccaccaatgtgagcccagcaaagcctaccacaaccgcatgcccatactctaaccccagcctgtgcacaaccacaccagcacccaggccccctacccctgcaccaacaatcgcctcccagcctctgtctctgcggccagaggcctgcagacccgccgccggcggagcagtgcacacacggggcctggactttgcctgtgatatctatatctgggccccactggctggaacatgtggcgtgctgctgctgtcactggtcattaccctgtactgtaagcgaggccggaagaaactgctgtatattttcaaacagccctttatgagacctgtgcagactacccaggaggaagacggctgcagctgtaggttccccgaggaagaggaaggcgggtgtgagctgagggtcaagtttagccgctccgcagatgcccctgcttaccagcaggggcagaatcagctgtataacgagctgaatctgggacggagagaggaatacgacgtgctggataaaaggcgcgggagagaccccgaaatgggaggcaagccacgacggaaaaacccccaggagggcctgtacaatgaactgcagaaggacaaaatggcagaggcctatagtgaaatcgggatgaagggagagagaaggcgcggcaaagggcacgatggcctgtaccaggggctgtctactgccaccaaggacacctatgatgctctgcatatgcaggcactgcctccaaggtga

SEQ ID NO: 33 - DNA, 1719 bp, artificial sequence
  2QR3
atggctctgcccgtcaccgctctgctgctgccactggccctgctgctgcacgccgccagacccggcggaggaggctcttgcccctacagcaaccccagcctgtgctctggcggcggcggcagcggaggcggcggctcccaggtgcagctgcagcagagcggccctggcctggtgaagccatcccagaccctgtctctgacatgcgccatcagcggcgactccgtgagctccaactctgccgcctggaattggatcagacagtccccatctaggggcctggagtggctgggaaggacctactatcggtccaagtggtacaacgactatgccgtgtctgtgaagagccgcatcaccatcaaccccgatacatccaagaatcagttctctctgcagctgaatagcgtgacccctgaggacacagccgtgtactattgcgccagagcctctatgaccggcggctacagctatggcgacgcctttgatatctggggccagggcacactggtgaccgtgtccggcggcggcggctctggaggaggaggaagcggaggaggaggatccgccatccgcatgacacagagcccttctagcctgagcgcctccgtgggcgatcgcgtgacaatcacctgtcgggcctctcagagcatctcctcttacctgaactggtatcagcagaagcccggcaaggcccctaagctgctgatctacgcagcaagctccctgcagagcggagtgccatcccggttctccggatctggaagcggaaccgacttttccctgacaatctctagcctgcagcctgaggattccgccacctactattgccagcagacatattctaccccactgacattcggccagggcacaaaggtggagatcaagggcagtggaggaggaggaagttgtccctactctaacccaagcctgtgcagtggaggaggaggaagtgaactgcctacccagggaacattcagcaacgtgtccaccaatgtgagcccagcaaagcctaccacaaccgcatgcccatactctaaccccagcctgtgcacaaccacaccagcacccaggccccctacccctgcaccaacaatcgcctcccagcctctgtctctgcggccagaggcctgcagacccgccgccggcggagcagtgcacacacggggcctggactttgcctgtgatatctatatctgggcaccactggccggaacatgtggcgtgctgctgctgtcactggtcattacactgtattgtaagcgaggccggaagaaactgctgtatattttcaaacagccctttatgagacctgtgcagactacccaggaggaagacggctgcagctgtaggttccccgaggaagaggaaggcgggtgtgagctgagggtcaagtttagccgctccgcagatgcccctgcttaccagcaggggcagaatcagctgtataacgagctgaatctgggacggagagaggaatacgacgtgctggataaaaggcgcgggagagaccccgaaatgggaggcaagccacgacggaaaaacccccaggagggcctgtacaatgaactgcagaaggacaaaatggcagaggcctatagtgaaatcgggatgaagggagagagaaggcgcggcaaagggcacgatggcctgtaccaggggctgtctactgccaccaaggacacctatgatgctctgcatatgcaggcactgcctccaaggtga

SEQ ID NO: 34 - DNA, 1707 bp, artificial sequence
  3QR3
atggctctgcccgtcaccgctctgctgctgccactggccctgctgctgcacgccgccagacccggcggaggaggctcttgcccctacagcaaccccagcctgtgctctggcggcggcggcagcggaggcggcggctcccaggtgcagctgcagcagagcggccctggcctggtggagccaagccagacactgtccctgacctgcgccatctctggcgacagcgtgagctccgattccgtggcctggaactggatcaggcagtctccaagccggggcctggagtggctgggcagaacatactataggtctacctggtacaatgactatgccggctccgtgaagtctcgcatcacaatcaaccccgataccagcaagaatcagttctccctgcagctgacatctgtgacccctgaggacacagccgtgtactattgcaccagatccaggcacaacacatttcggggaatggacgtgtggggacagggaaccacagtgaccgtgagcggaggaggaggatccggcggaggaggctctggaggaggaggaagcgacatcgtgatgacccagagcccttctagcctgtccgcctctgtgggcgatagagtgacaatcacctgtagggcctcccagaccatctcctcttacctgaactggtatcagcagaagcccggcaaggcccctaagctgctgatctacgacgcaagctccctgcagtctggagtgccaagcagattcagcggctccggctctggcaccgactttacactgaccatcaattccctgcagcctgaggatttcgccacatactattgccagcagtcttataccacaccaatcacatttggccagggcacccgcctggagatcaagggaagcggcggcggcggctcatgcccttattcaaacccatctctgtgctcaggaggaggaggaagcgaactgcctactcagggaacattcagcaacgtgtccaccaatgtgagcccagcaaagcctaccacaaccgcatgcccatactctaaccccagcctgtgcacaaccacaccagcacccaggccccctacccctgcaccaacaatcgcctcccagcctctgtctctgcggccagaggcctgcagacccgccgccggcggagcagtgcacacacggggcctggactttgcctgtgatatctatatctgggcaccactggctggaacatgtggcgtgctgctgctgtcactggtcattacactgtattgcaagcgaggccggaagaaactgctgtatattttcaaacagccctttatgagacctgtgcagactacccaggaggaagacggctgcagctgtaggttccccgaggaagaggaaggcgggtgtgagctgagggtcaagtttagccgctccgcagatgcccctgcttaccagcaggggcagaatcagctgtataacgagctgaatctgggacggagagaggaatacgacgtgctggataaaaggcgcgggagagaccccgaaatgggaggcaagccacgacggaaaaacccccaggagggcctgtacaatgaactgcagaaggacaaaatggcagaggcctatagtgaaatcgggatgaagggagagagaaggcgcggcaaagggcacgatggcctgtaccaggggctgtctactgccaccaaggacacctatgatgctctgcatatgcaggcactgcctccaaggtga

SEQ ID NO: 35 - DNA, 1707 bp, artificial sequence
  4QR3
atggctctgcccgtcaccgctctgctgctgccactggccctgctgctgcacgccgccagacccggcggaggaggctcttgcccctacagcaaccccagcctgtgctctggcggcggcggcagcggaggcggcggctcccaggtgcagctgcagcagagcggccctggcctggtggagccaagccagacactgtccctgacctgcgccatctctggcgacagcgtgagctccaacagcgccgcatggaattggatcaggcagtccccatctcggggcctggagtggctgggcagaacatactataggtccacctggtacaacgactatgccggctccgtgaagtctcgcatcacaatcaaccccgataccagcaagaatcagttctccctgcagctgacatctgtgacccctgaggacacagccgtgtactattgcaccagaagcaggcacaatacatttcggggaatggacgtgtggggacagggcacactggtgaccgtgagcggaggaggaggatccggcggaggaggctctggcggcggcggcagcgacatccagctgacccagtccccttctagcctgagcgcctccgtgggcgatagagtgacaatcacctgtagggcctctcagagcatctcctcttacctgaactggtatcagcagaagcccggcaaggcccctaagctgctgatctacgcagcaagctccctgcagtctggagtgccaagcagattctccggctctggcagcggcaccgactttacactgaccatctctagcctgcagcctgaggatttcgccacatactattgccagcagtcctattctacaccactgacctttggcggcggcaccaaggtggagatcaagggaagcggcggcggcggaagttgtccatattcaaacccaagtctgtgcagcggcggaggaggaagcgaactgcctactcagggaaccttcagcaacgtgtccaccaatgtgagcccagcaaagcctaccacaaccgcatgcccatactctaaccccagcctgtgcacaaccacaccagcacccaggccccctacccctgcaccaacaatcgcctcccagcctctgtctctgcggccagaggcctgcagacccgccgccggcggagcagtgcacacacggggcctggactttgcctgtgatatctatatctgggcaccactggccggaacatgtggcgtgctgctgctgtcactggtcattacactgtactgtaagcgaggccggaagaaactgctgtatattttcaaacagccctttatgagacctgtgcagactacccaggaggaagacggctgcagctgtaggttccccgaggaagaggaaggcgggtgtgagctgagggtcaagtttagccgctccgcagatgcccctgcttaccagcaggggcagaatcagctgtataacgagctgaatctgggacggagagaggaatacgacgtgctggataaaaggcgcgggagagaccccgaaatgggaggcaagccacgacggaaaaacccccaggagggcctgtacaatgaactgcagaaggacaaaatggcagaggcctatagtgaaatcgggatgaagggagagagaaggcgcggcaaagggcacgatggcctgtaccaggggctgtctactgccaccaaggacacctatgatgctctgcatatgcaggcactgcctccaaggtga

SEQ ID NO: 36 - DNA, 1695 bp, artificial sequence
  5QR3
atggctctgcccgtcaccgctctgctgctgccactggccctgctgctgcacgccgccagacccggcggaggaggctcttgcccctacagcaaccccagcctgtgctctggcggcggcggcagcggaggcggcggctcccaggtgcagctgcagcagagcggccctggcctggtggagccaagccagaccctgtccctgacatgcgccatctctggcgacagcgtgagctccgattctgtggcctggaactggatcaggcagagcccaagccggggcctggagtggctgggcagaacctactataggtccacatggtacaatgactatgccggctccgtgaagtctcggatcaccatcaaccccgatacatccaagaatcagttctctctgcagctgaacagcgtgacccctgaggacacagccgtgtactattgcgccagagacaggaatggcatggacgtgtggggccagggaaccatggtgacagtgtccggaggaggcggctctggaggaggaggaagcggaggaggaggatccgacatcgtgatgacccagagcccttctagcctgtctgccagcgtgggcgatagagtgacaatcacctgtagggcctcccagtctatctcctcttacctgaactggtatcagcagaagcccggcaaggcccctaagctgctgatctacgatgcctctaatctggagacaggcgtgccaagcagattcagcggctccggctctggcacagacttcaccttcaccatcacatccctgcagcctgaggatttcgccacctactattgccagcagtcttataccacaccactgacctttggcggcggcacaaaggtggagatcaagggaagcggaggaggaggaagttgtccctattcaaatccatcactgtgcagcggaggaggaggaagcgaactgcctactcagggaaccttcagcaacgtgtccaccaatgtgagcccagcaaagcctaccacaaccgcatgcccatactctaaccccagcctgtgcacaaccacaccagcacccaggccccctacccctgcaccaacaatcgcctcccagcctctgtctctgcggccagaggcctgcagacccgccgccggcggagcagtgcacacacggggcctggactttgcctgtgatatctatatctgggcaccactggctggaacatgcggcgtgctgctgctgtcactggtcatcacactgtactgtaagcgaggccggaagaaactgctgtatattttcaaacagccctttatgagacctgtgcagactacccaggaggaagacggctgcagctgtaggttccccgaggaagaggaaggcgggtgtgagctgagggtcaagtttagccgctccgcagatgcccctgcttaccagcaggggcagaatcagctgtataacgagctgaatctgggacggagagaggaatacgacgtgctggataaaaggcgcgggagagaccccgaaatgggaggcaagccacgacggaaaaacccccaggagggcctgtacaatgaactgcagaaggacaaaatggcagaggcctatagtgaaatcgggatgaagggagagagaaggcgcggcaaagggcacgatggcctgtaccaggggctgtctactgccaccaaggacacctatgatgctctgcatatgcaggcactgcctccaaggtga

SEQ ID NO: 37 - DNA, 1704 bp, artificial sequence
  6QR3
atggctctgcccgtcaccgctctgctgctgccactggccctgctgctgcacgccgccagacccggcggaggaggctcttgcccctacagcaaccccagcctgtgctctggcggcggcggcagcggaggcggcggctcccaggtgcagctgcagcagtccggcccaggcctggtgaagccatcccagacactgtctctgacctgcgccatcagcggcgactccgtgagctcctctagcgccgcctggaactggatcagacagtctcctagcaggggcctggagtggctgggaaggacctactatcggtccgcctggtacaatgactatgccgtgtctgtgaagagcagaatcacaatcaaccccgatacctccaagaatcagttctctctgcagctgaacagcgtgacacctgaggataccgccgtgtactattgcgccagagagagcgtgctgctggacggaatggacgtgtggggaaggggaaccacagtgacagtgtccggaggaggcggctctggaggaggaggaagcggaggaggaggatccgccatcaggatgacacagtccccatctaccctgagcgcctccgtgggcgaccgcgtgacaatcacctgtcgggcctctcagagcatctccacctacctgaattggtatcagcagaaggccggcaaggccccaagactgctgatccacgatgcatcctctctgcagagcggagtgccatccaggttctctggaagcggatccggcacagactttacactgaccatcagctccctgcagcctgaggatttcgccacctactattgccagcagtcttacagcacaccactgacctttggcggcggcacaaaggtggagatcaagggaagcgggggaggaggatcttgcccatattcaaacccatcactgtgctcaggaggaggaggaagcgaactgcctactcagggaactttcagcaacgtgtccaccaatgtgagcccagcaaagcctaccacaaccgcatgcccatactctaaccccagcctgtgcacaaccacaccagcacccaggccccctacccctgcaccaacaatcgcctcccagcctctgtctctgcggccagaggcctgcagacccgccgccggcggagcagtgcacacacggggcctggactttgcctgtgatatctatatctgggcaccactggccggaacatgtggcgtgctgctgctgtcactggtcattacactgtactgtaagcgaggccggaagaaactgctgtatattttcaaacagccctttatgagacctgtgcagactacccaggaggaagacggctgcagctgtaggttccccgaggaagaggaaggcgggtgtgagctgagggtcaagtttagccgctccgcagatgcccctgcttaccagcaggggcagaatcagctgtataacgagctgaatctgggacggagagaggaatacgacgtgctggataaaaggcgcgggagagaccccgaaatgggaggcaagccacgacggaaaaacccccaggagggcctgtacaatgaactgcagaaggacaaaatggcagaggcctatagtgaaatcgggatgaagggagagagaaggcgcggcaaagggcacgatggcctgtaccaggggctgtctactgccaccaaggacacctatgatgctctgcatatgcaggcactgcctccaaggtga

SEQ ID NO: 38 - DNA, 1725 bp, artificial sequence
  7QR3
atggctctgcccgtcaccgctctgctgctgccactggccctgctgctgcacgccgccagacccggcggaggaggctcttgcccctacagcaaccccagcctgtgctctggcggcggcggcagcggaggcggcggctcccaggtgcagctgcagcagagcggccctggcctggtgcagccatcccagacactgtctctgacctgcgtgatcagcggcgactccgtgagctccaactctgccacatggaattggatcagacagagcccatccaggggcctggagtggctgggacgcacctactatcggagcaagtggtacaacgactatgccgtgtctgtgaagagcagaatcacaatcaaccccgatacctctaagaatcagttcagcctgcagctgaattccgtgacacctgaggataccgccgtgtactattgcgccagggacggcgatggaggaagctactatgactactattactatggcatggacgtgtggggccagggcaccacagtgacagtgtctggaggaggaggaagcggaggaggaggatccggcggcggcggctctgacatccagctgacacagtccccttctagcctgtctaccagcgtgggcgatcgcgtgacaatcacctgtcgggcctcccagtctatcagcacctacctgaactggtatcagcagaagcccggcaaggcccctaagctgctgatctacgcagcaagcaatctgcagtccggagtgccatctcgcttctccggctctggcagcggcacagactttacactgaccatctcctctctgcagcctgaggatttcgccacctacttttgccagcagtcctataccacaccaatcacattcggccagggcaccagactggagatcaagggaagtggaggaggaggaagttgcccttactctaacccaagtctgtgctcaggaggcggaggaagcgaactgcctactcagggaacattcagcaacgtgtccaccaatgtgagcccagcaaagcctaccacaaccgcatgcccatactctaaccccagcctgtgcacaaccacaccagcacccaggccccctacccctgcaccaacaatcgcctcccagcctctgtctctgcggccagaggcctgcagacccgccgccggcggagcagtgcacacacggggcctggactttgcctgtgatatctatatctgggcaccactggctggaacatgcggagtgctgctgctgtcactggtcattacactgtactgtaagcgaggccggaagaaactgctgtatattttcaaacagccctttatgagacctgtgcagactacccaggaggaagacggctgcagctgtaggttccccgaggaagaggaaggcgggtgtgagctgagggtcaagtttagccgctccgcagatgcccctgcttaccagcaggggcagaatcagctgtataacgagctgaatctgggacggagagaggaatacgacgtgctggataaaaggcgcgggagagaccccgaaatgggaggcaagccacgacggaaaaacccccaggagggcctgtacaatgaactgcagaaggacaaaatggcagaggcctatagtgaaatcgggatgaagggagagagaaggcgcggcaaagggcacgatggcctgtaccaggggctgtctactgccaccaaggacacctatgatgctctgcatatgcaggcactgcctccaaggtga

SEQ ID NO: 39 - DNA, 1695 bp, artificial sequence
  8QR3
atggctctgcccgtcaccgctctgctgctgccactggccctgctgctgcacgccgccagacccggcggaggaggctcttgcccctacagcaaccccagcctgtgctctggcggcggcggcagcggaggcggcggctcccaggtgcagctgcagcagtccggccctggcctggtgaagccatctcagacactgagcctgacctgcgccatctccggcgactctgtgagctccaactccgccgcctggaattggatcagacagagcccatccaggggcctggagtggctgggacgcacctactatcggagcgcctggtacaacgactatgccgtgagcgtgaagtccagaatcacaatcaaccccgatacctctaagaatcagttcagcctgcagctgtctagcgtgacacctgaggataccgccgtgtactattgcgccagggacgtggagggctttgattactggggccagggcacactggtgaccgtgtccggcggcggcggctctggaggaggaggaagcggaggaggaggatccgacatcgtgatgacacagaccccttcctctctgtctgccagcgtgggcgatcgcgtgacaatcacctgtcgggcctcccagtctatcagctcctacctgaattggtatcagcagaagcccggcaaggcccctaagctgctgatctacgcagcatctagcctgcagtccggagtgccatctcgcttcagcggatccggctctggcacagactttacactgaccatctcctctctgcagcctgaggatttcgccacctactattgccagcagagctattccacaccaatcacctttggccagggcacaagactggagatcaagggaagcgggggaggaggatcatgtccatactctaacccatcactgtgctctggaggaggaggaagcgaactgcctactcagggaaccttcagcaacgtgtccaccaatgtgagcccagcaaagcctaccacaaccgcatgcccatactctaaccccagcctgtgcacaaccacaccagcacccaggccccctacccctgcaccaacaatcgcctcccagcctctgtctctgcggccagaggcctgcagacccgccgccggcggagcagtgcacacacggggcctggactttgcctgtgatatctatatctgggcaccactggctggaacatgcggcgtgctgctgctgtcactggtcattacactgtattgtaagcgaggccggaagaaactgctgtatattttcaaacagccctttatgagacctgtgcagactacccaggaggaagacggctgcagctgtaggttccccgaggaagaggaaggcgggtgtgagctgagggtcaagtttagccgctccgcagatgcccctgcttaccagcaggggcagaatcagctgtataacgagctgaatctgggacggagagaggaatacgacgtgctggataaaaggcgcgggagagaccccgaaatgggaggcaagccacgacggaaaaacccccaggagggcctgtacaatgaactgcagaaggacaaaatggcagaggcctatagtgaaatcgggatgaagggagagagaaggcgcggcaaagggcacgatggcctgtaccaggggctgtctactgccaccaaggacacctatgatgctctgcatatgcaggcactgcctccaaggtga

SEQ ID NO: 40 - DNA, 1710 bp, artificial sequence
  9QR3
atggctctgcccgtcaccgctctgctgctgccactggccctgctgctgcacgccgccagacccggcggaggaggctcttgcccctacagcaaccccagcctgtgctctggcggcggcggcagcggaggcggcggctcccaggtgcagctgcagcagagcggccccggcctggtgaagcctagccagacactgtccctgacctgcgcaatctccggcgacagcgtgtccggaaacagggccacatggaattggatcagacagtctccaagcaggggcctggagtggctgggaaggacctactatcggtccgcctggtacaacgactatgccgtgtctgtgaagggccgcatcacattcaacccagataccagcaagaatcagttttccctgcagctgaattctgtgacacccgaggataccgccgtgtactattgcgccagaggcgagagcggagcagcagcagacgccttcgatatctggggccagggcaccacagtgacagtgagcggaggaggaggatccggcggaggaggctctggcggcggcggcagcgacatccagctgacccagagcccaccttccctgtctgccagcgtgggcgatcgcgtgacaatcacctgtcgggcctcccagtctatcagctcctacctgaactggtatcagcagaagccaggcaaggcccccaagctgctgatctacgcagcatctagcctgcagtctggagtgccaagcagattcagcggatccggattcggcacagactttacactgaccatctcctctctgcagcccgaggatttcgccacctactattgccagcagtcttatagcacacctcagacctttggccagggcaccaaggtggacatcaagggaagtggaggaggaggaagttgtccctactcaaacccatctctgtgctcaggaggaggaggaagtgaactgcctactcagggaacattcagcaacgtgtccaccaatgtgagcccagcaaagcctaccacaaccgcatgcccatactctaaccccagcctgtgcacaaccacaccagcacccaggccccctacccctgcaccaacaatcgcctcccagcctctgtctctgcggccagaggcctgcagacccgccgccggcggagcagtgcacacacggggcctggactttgcctgtgatatctatatctgggcaccactggccggaacatgtggcgtgctgctgctgtcactggtcattacactgtactgtaagcgaggccggaagaaactgctgtatattttcaaacagccctttatgagacctgtgcagactacccaggaggaagacggctgcagctgtaggttccccgaggaagaggaaggcgggtgtgagctgagggtcaagtttagccgctccgcagatgcccctgcttaccagcaggggcagaatcagctgtataacgagctgaatctgggacggagagaggaatacgacgtgctggataaaaggcgcgggagagaccccgaaatgggaggcaagccacgacggaaaaacccccaggagggcctgtacaatgaactgcagaaggacaaaatggcagaggcctatagtgaaatcgggatgaagggagagagaaggcgcggcaaagggcacgatggcctgtaccaggggctgtctactgccaccaaggacacctatgatgctctgcatatgcaggcactgcctccaaggtga

SEQ ID NO: 41 - DNA, 1710 bp, artificial sequence
  10QR3
atggctctgcccgtcaccgctctgctgctgccactggccctgctgctgcacgccgccagacccggcggaggaggctcttgcccctacagcaaccccagcctgtgctctggcggcggcggcagcggaggcggcggctcccaggtgcagctggtgcagagcggagcagaggtgaagaagcctggcgccagcgtgaaggtgtcctgcaaggcctctggctacacattcaccagctactatatgcactgggtgcggcaggcccctggccagggcctggagtggatgggcatcatcaacccatccggcggctccacctcttacgcccagaagtttcagggcagagtgacaatgaccagggacacaagcacctccacagtgtatatggagctgagctccctgagatccgaggatacagccgtgtactattgcgccagggaggactctggaagcggagccttcgatatctggggccagggcaccctggtgacagtgtctggaggaggaggaagcggaggaggaggatccggcggcggcggctctgagatcgtgctgacccagtctccactgagcctgccagtgacacctggcgagccagcctccatctcttgtcgctctagccggtccctgctgtcttaccacggctacaattatctggactggtatctgcagaagccaggccagagcccccagctgctgatcttcgtgggatccaacagggcccctggcgtgcctgaccggttcagcggatccggatctggaaccgacttcaccctgaacatctctagagtggaggccgaggatgtgggcgtgtactattgcatgcagagcctgcagaccccaagaacatttggccagggcaccaaggtggagatcaagggaagcggcggaggcggaagttgtccctactcaaacccaagtctgtgctcaggaggaggaggaagcgaactgcctactcagggaacattcagcaacgtgtccaccaatgtgagcccagcaaagcctaccacaaccgcatgcccatactctaaccccagcctgtgcacaaccacaccagcacccaggccccctacccctgcaccaacaatcgcctcccagcctctgtctctgcggccagaggcctgcagacccgccgccggcggagcagtgcacacacggggcctggactttgcctgtgatatctatatctgggcaccactggccggaacatgcggagtcctgctgctgtcactggtcattacactgtactgtaagcgaggccggaagaaactgctgtatattttcaaacagccctttatgagacctgtgcagactacccaggaggaagacggctgcagctgtaggttccccgaggaagaggaaggcgggtgtgagctgagggtcaagtttagccgctccgcagatgcccctgcttaccagcaggggcagaatcagctgtataacgagctgaatctgggacggagagaggaatacgacgtgctggataaaaggcgcgggagagaccccgaaatgggaggcaagccacgacggaaaaacccccaggagggcctgtacaatgaactgcagaaggacaaaatggcagaggcctatagtgaaatcgggatgaagggagagagaaggcgcggcaaagggcacgatggcctgtaccaggggctgtctactgccaccaaggacacctatgatgctctgcatatgcaggcactgcctccaaggtga

SEQ ID NO: 42 - DNA, 1587 bp, artificial sequence
  CAR 4 R2
atggctctgcccgtcaccgctctgctgctgcccctggccctgctgctgcacgccgcccggcctcaggtgcagctgcagcagagcggccctggcctggtggagccaagccagacactgtccctgacctgcgccatctctggcgacagcgtgagctccaacagcgccgcatggaattggatcaggcagtccccatctcggggcctggagtggctgggcagaacatactataggtccacctggtacaacgactatgccggctccgtgaagtctcgcatcacaatcaaccccgataccagcaagaatcagttctccctgcagctgacatctgtgacccctgaggacacagccgtgtactattgcaccagaagcaggcacaatacatttcggggaatggacgtgtggggacagggcacactggtgaccgtgagcggaggaggaggatccggcggaggaggctctggcggcggcggcagcgacatccagctgacccagtccccttctagcctgagcgcctccgtgggcgatagagtgacaatcacctgtagggcctctcagagcatctcctcttacctgaactggtatcagcagaagcccggcaaggcccctaagctgctgatctacgcagcaagctccctgcagtctggagtgccaagcagattctccggctctggcagcggcaccgactttacactgaccatctctagcctgcagcctgaggatttcgccacatactattgccagcagtcctattctacaccactgacctttggcggcggcaccaaggtggagatcaagtctgaccccggaagtggcggcggcggaagttgcccttattcaaatccatccctgtgctctggcggcggaggaagttgtccttatagcaaccccagcctgtgctccggaggaggaggcagcaccacaaccccagcacccaggccccctacacctgcaccaaccatcgcctctcagccactgagcctgcggcctgaggcctgcagaccagccgccggcggagcagtgcacacacggggcctggacttcgcctgtgatatctacatctgggcaccactggccggaacatgtggcgtgctgctgctgtcactggtcattacactgtactgtaagcgaggccggaagaaactgctgtatattttcaaacagccctttatgagacctgtgcagactacccaggaggaagacggctgcagctgtaggttccccgaggaagaggaaggcgggtgtgagctgagggtcaagtttagccgctccgcagatgcccctgcttaccagcaggggcagaatcagctgtataacgagctgaatctgggacggagagaggaatacgacgtgctggataaaaggcgcgggagagaccccgaaatgggaggcaagccacgacggaaaaacccccaggagggcctgtacaatgaactgcagaaggacaaaatggcagaggcctatagtgaaatcgggatgaagggagagagaaggcgcggcaaagggcacgatggcctgtaccaggggctgtctactgccaccaaggacacctatgatgctctgcatatgcaggcactgcctccaaggtga

SEQ ID NO: 43 - DNA, 1605 bp, artificial sequence
  CAR7_R2
atggctctgcccgtcaccgctctgctgctgcccctggccctgctgctgcacgccgcccggcctcaggtgcagctgcagcagagcggccctggcctggtgcagccatcccagacactgtctctgacctgcgtgatcagcggcgactccgtgagctccaactctgccacatggaattggatcagacagagcccatccaggggcctggagtggctgggacgcacctactatcggagcaagtggtacaacgactatgccgtgtctgtgaagagcagaatcacaatcaaccccgatacctctaagaatcagttcagcctgcagctgaattccgtgacacctgaggataccgccgtgtactattgcgccagggacggcgatggaggaagctactatgactactattactatggcatggacgtgtggggccagggcaccacagtgacagtgtctggaggaggaggaagcggaggaggaggatccggcggcggcggctctgacatccagctgacacagtccccttctagcctgtctaccagcgtgggcgatcgcgtgacaatcacctgtcgggcctcccagtctatcagcacctacctgaactggtatcagcagaagcccggcaaggcccctaagctgctgatctacgcagcaagcaatctgcagtccggagtgccatctcgcttctccggctctggcagcggcacagactttacactgaccatctcctctctgcagcctgaggatttcgccacctacttttgccagcagtcctataccacaccaatcacattcggccagggcaccagactggagatcaagagcgaccccggcagtggaggaggaggctcttgtccctactctaacccatctctgtgcagtggcggaggaggctcttgcccttattccaaccccagcctgtgctccggaggaggaggcagcaccacaaccccagcacccaggccccctacacctgcaccaaccatcgcctctcagccactgagcctgcggcctgaggcctgcagaccagccgccggcggagcagtgcacacacggggcctggacttcgcctgtgatatctacatctgggcaccactggccggaacatgtggcgtgctgctgctgtcactggtcattacactgtactgtaagcgaggccggaagaaactgctgtatattttcaaacagccctttatgagacctgtgcagactacccaggaggaagacggctgcagctgtaggttccccgaggaagaggaaggcgggtgtgagctgagggtcaagtttagccgctccgcagatgcccctgcttaccagcaggggcagaatcagctgtataacgagctgaatctgggacggagagaggaatacgacgtgctggataaaaggcgcgggagagaccccgaaatgggaggcaagccacgacggaaaaacccccaggagggcctgtacaatgaactgcagaaggacaaaatggcagaggcctatagtgaaatcgggatgaagggagagagaaggcgcggcaaagggcacgatggcctgtaccaggggctgtctactgccaccaaggacacctatgatgctctgcatatgcaggcactgcctccaaggtga

SEQ ID NO: 44 - DNA, 1590 bp, artificial sequence
  CAR9 R2
atggctctgcccgtcaccgctctgctgctgcccctggccctgctgctgcacgccgcccggcctcaggtgcagctgcagcagagcggccccggcctggtgaagcctagccagacactgtccctgacctgcgcaatctccggcgacagcgtgtccggaaacagggccacatggaattggatcagacagtctccaagcaggggcctggagtggctgggaaggacctactatcggtccgcctggtacaacgactatgccgtgtctgtgaagggccgcatcacattcaacccagataccagcaagaatcagttttccctgcagctgaattctgtgacacccgaggataccgccgtgtactattgcgccagaggcgagagcggagcagcagcagacgccttcgatatctggggccagggcaccacagtgacagtgagcggaggaggaggatccggcggaggaggctctggcggcggcggcagcgacatccagctgacccagagcccaccttccctgtctgccagcgtgggcgatcgcgtgacaatcacctgtcgggcctcccagtctatcagctcctacctgaactggtatcagcagaagccaggcaaggcccccaagctgctgatctacgcagcatctagcctgcagtctggagtgccaagcagattcagcggatccggattcggcacagactttacactgaccatctcctctctgcagcccgaggatttcgccacctactattgccagcagtcttatagcacacctcagacctttggccagggcaccaaggtggacatcaagagcgaccccggaagcggaggaggaggaagttgtccctactcaaaccctagcctgtgtagcggcggcggaggatcttgtccctattctaaccccagcctgtgctccggaggaggaggcagcaccacaaccccagcacccaggccccctacacctgcaccaaccatcgcctctcagccactgagcctgcggcctgaggcctgcagaccagccgccggcggagcagtgcacacacggggcctggacttcgcctgtgatatctacatctgggcaccactggctggaacatgcggagtgctgctgctgtcactggtcattacactgtactgtaagcgaggccggaagaaactgctgtatattttcaaacagccctttatgagacctgtgcagactacccaggaggaagacggctgcagctgtaggttccccgaggaagaggaaggcgggtgtgagctgagggtcaagtttagccgctccgcagatgcccctgcttaccagcaggggcagaatcagctgtataacgagctgaatctgggacggagagaggaatacgacgtgctggataaaaggcgcgggagagaccccgaaatgggaggcaagccacgacggaaaaacccccaggagggcctgtacaatgaactgcagaaggacaaaatggcagaggcctatagtgaaatcgggatgaagggagagagaaggcgcggcaaagggcacgatggcctgtaccaggggctgtctactgccaccaaggacacctatgatgctctgcatatgcaggcactgcctccaaggtga

SEQ ID NO: 45 - DNA, 1590 bp, artificial sequence
  CAR10R2
atggctctgcccgtcaccgctctgctgctgcccctggccctgctgctgcacgccgcccggcctcaggtgcagctggtgcagagcggagcagaggtgaagaagcctggcgccagcgtgaaggtgtcctgcaaggcctctggctacacattcaccagctactatatgcactgggtgcggcaggcccctggccagggcctggagtggatgggcatcatcaacccatccggcggctccacctcttacgcccagaagtttcagggcagagtgacaatgaccagggacacaagcacctccacagtgtatatggagctgagctccctgagatccgaggatacagccgtgtactattgcgccagggaggactctggaagcggagccttcgatatctggggccagggcaccctggtgacagtgtctggaggaggaggaagcggaggaggaggatccggcggcggcggctctgagatcgtgctgacccagtctccactgagcctgccagtgacacctggcgagccagcctccatctcttgtcgctctagccggtccctgctgtcttaccacggctacaattatctggactggtatctgcagaagccaggccagagcccccagctgctgatcttcgtgggatccaacagggcccctggcgtgcctgaccggttcagcggatccggatctggaaccgacttcaccctgaacatctctagagtggaggccgaggatgtgggcgtgtactattgcatgcagagcctgcagaccccaagaacatttggccagggcaccaaggtggagatcaagagcgaccccggaagcggcggaggaggaagttgtccctattctaacccatctctgtgcagcggcggcggaggaagttgtccttattcaaaccccagcctgtgctccggaggaggaggcagcaccacaaccccagcacccaggccccctacacctgcaccaaccatcgcctctcagccactgagcctgcggcctgaggcctgcagaccagccgccggcggagcagtgcacacacggggcctggacttcgcctgtgatatctacatctgggcaccactggctggaacatgcggcgtgctgctgctgtcactggtcattacactgtactgtaagcgaggccggaagaaactgctgtatattttcaaacagccctttatgagacctgtgcagactacccaggaggaagacggctgcagctgtaggttccccgaggaagaggaaggcgggtgtgagctgagggtcaagtttagccgctccgcagatgcccctgcttaccagcaggggcagaatcagctgtataacgagctgaatctgggacggagagaggaatacgacgtgctggataaaaggcgcgggagagaccccgaaatgggaggcaagccacgacggaaaaacccccaggagggcctgtacaatgaactgcagaaggacaaaatggcagaggcctatagtgaaatcgggatgaagggagagagaaggcgcggcaaagggcacgatggcctgtaccaggggctgtctactgccaccaaggacacctatgatgctctgcatatgcaggcactgcctccaaggtga

SEQ ID NO: 46 - protein, 487 aa, artificial sequence
  CAR 1
MALPVTALLLPLALLLHAARPQVQLQQSGPGLVKPSQTLSLTCAISGDSVSSNSAAWNWIRQSPSRGLEWLGRTYYRSTWYNDYAVSVKSRITINPDTSKNQFSLQLNSVTPEDTAVYYCAREVSGTSAFDIWGQGTMVTVSGGGGSGGGGSGGGGSDIQMTQSPSSLSASVGDRVTITCRASQSISSYLNWYQQKPGKAPKLLIYAASSLQSGVPSRFSGSGSGTDFTLTISSLQPEDFATYYCQQSYSTPLTFGGGTKLEIKTTTPAPRPPTPAPTIASQPLSLRPEACRPAAGGAVHTRGLDFACDIYIWAPLAGTCGVLLLSLVITLYCKRGRKKLLYIFKQPFMRPVQTTQEEDGCSCRFPEEEEGGCELRVKFSRSADAPAYQQGQNQLYNELNLGRREEYDVLDKRRGRDPEMGGKPRRKNPQEGLYNELQKDKMAEAYSEIGMKGERRRGKGHDGLYQGLSTATKDTYDALHMQALPPR

SEQ ID NO: 47 - protein, 492 aa, artificial sequence
  CAR 2
MALPVTALLLPLALLLHAARPQVQLQQSGPGLVKPSQTLSLTCAISGDSVSSNSAAWNWIRQSPSRGLEWLGRTYYRSKWYNDYAVSVKSRITINPDTSKNQFSLQLNSVTPEDTAVYYCARASMTGGYSYGDAFDIWGQGTLVTVSGGGGSGGGGSGGGGSAIRMTQSPSSLSASVGDRVTITCRASQSISSYLNWYQQKPGKAPKLLIYAASSLQSGVPSRFSGSGSGTDFSLTISSLQPEDSATYYCQQTYSTPLTFGQGTKVEIKTTTPAPRPPTPAPTIASQPLSLRPEACRPAAGGAVHTRGLDFACDIYIWAPLAGTCGVLLLSLVITLYCKRGRKKLLYIFKQPFMRPVQTTQEEDGCSCRFPEEEEGGCELRVKFSRSADAPAYQQGQNQLYNELNLGRREEYDVLDKRRGRDPEMGGKPRRKNPQEGLYNELQKDKMAEAYSEIGMKGERRRGKGHDGLYQGLSTATKDTYDALHMQALPPR

SEQ ID NO: 48 - protein, 488 aa, artificial sequence
  CAR 3
MALPVTALLLPLALLLHAARPQVQLQQSGPGLVEPSQTLSLTCAISGDSVSSDSVAWNWIRQSPSRGLEWLGRTYYRSTWYNDYAGSVKSRITINPDTSKNQFSLQLTSVTPEDTAVYYCTRSRHNTFRGMDVWGQGTTVTVSGGGGSGGGGSGGGGSDIVMTQSPSSLSASVGDRVTITCRASQTISSYLNWYQQKPGKAPKLLIYDASSLQSGVPSRFSGSGSGTDFTLTINSLQPEDFATYYCQQSYTTPITFGQGTRLEIKTTTPAPRPPTPAPTIASQPLSLRPEACRPAAGGAVHTRGLDFACDIYIWAPLAGTCGVLLLSLVITLYCKRGRKKLLYIFKQPFMRPVQTTQEEDGCSCRFPEEEEGGCELRVKFSRSADAPAYQQGQNQLYNELNLGRREEYDVLDKRRGRDPEMGGKPRRKNPQEGLYNELQKDKMAEAYSEIGMKGERRRGKGHDGLYQGLSTATKDTYDALHMQALPPR

SEQ ID NO: 49 - protein, 488 aa, artificial sequence
  CAR 4
MALPVTALLLPLALLLHAARPQVQLQQSGPGLVEPSQTLSLTCAISGDSVSSNSAAWNWIRQSPSRGLEWLGRTYYRSTWYNDYAGSVKSRITINPDTSKNQFSLQLTSVTPEDTAVYYCTRSRHNTFRGMDVWGQGTLVTVSGGGGSGGGGSGGGGSDIQLTQSPSSLSASVGDRVTITCRASQSISSYLNWYQQKPGKAPKLLIYAASSLQSGVPSRFSGSGSGTDFTLTISSLQPEDFATYYCQQSYSTPLTFGGGTKVEIKTTTPAPRPPTPAPTIASQPLSLRPEACRPAAGGAVHTRGLDFACDIYIWAPLAGTCGVLLLSLVITLYCKRGRKKLLYIFKQPFMRPVQTTQEEDGCSCRFPEEEEGGCELRVKFSRSADAPAYQQGQNQLYNELNLGRREEYDVLDKRRGRDPEMGGKPRRKNPQEGLYNELQKDKMAEAYSEIGMKGERRRGKGHDGLYQGLSTATKDTYDALHMQALPPR

SEQ ID NO: 50 - protein, 484 aa, artificial sequence
  CAR 5
MALPVTALLLPLALLLHAARPQVQLQQSGPGLVEPSQTLSLTCAISGDSVSSDSVAWNWIRQSPSRGLEWLGRTYYRSTWYNDYAGSVKSRITINPDTSKNQFSLQLNSVTPEDTAVYYCARDRNGMDVWGQGTMVTVSGGGGSGGGGSGGGGSDIVMTQSPSSLSASVGDRVTITCRASQSISSYLNWYQQKPGKAPKLLIYDASNLETGVPSRFSGSGSGTDFTFTITSLQPEDFATYYCQQSYTTPLTFGGGTKVEIKTTTPAPRPPTPAPTIASQPLSLRPEACRPAAGGAVHTRGLDFACDIYIWAPLAGTCGVLLLSLVITLYCKRGRKKLLYIFKQPFMRPVQTTQEEDGCSCRFPEEEEGGCELRVKFSRSADAPAYQQGQNQLYNELNLGRREEYDVLDKRRGRDPEMGGKPRRKNPQEGLYNELQKDKMAEAYSEIGMKGERRRGKGHDGLYQGLSTATKDTYDALHMQALPPR

SEQ ID NO: 51 - protein, 487 aa, artificial sequence
  CAR 6-8
MALPVTALLLPLALLLHAARPQVQLQQSGPGLVKPSQTLSLTCAISGDSVSSSSAAWNWIRQSPSRGLEWLGRTYYRSAWYNDYAVSVKSRITINPDTSKNQFSLQLNSVTPEDTAVYYCARESVLLDGMDVWGRGTTVTVSGGGGSGGGGSGGGGSAIRMTQSPSTLSASVGDRVTITCRASQSISTYLNWYQQKAGKAPRLLIHDASSLQSGVPSRFSGSGSGTDFTLTISSLQPEDFATYYCQQSYSTPLTFGGGTKVEIKTTTPAPRPPTPAPTIASQPLSLRPEACRPAAGGAVHTRGLDFACDIYIWAPLAGTCGVLLLSLVITLYCKRGRKKLLYIFKQPFMRPVQTTQEEDGCSCRFPEEEEGGCELRVKFSRSADAPAYQQGQNQLYNELNLGRREEYDVLDKRRGRDPEMGGKPRRKNPQEGLYNELQKDKMAEAYSEIGMKGERRRGKGHDGLYQGLSTATKDTYDALHMQALPPR

SEQ ID NO: 52 - protein, 494 aa, artificial sequence
  CAR 7 9
MALPVTALLLPLALLLHAARPQVQLQQSGPGLVQPSQTLSLTCVISGDSVSSNSATWNWIRQSPSRGLEWLGRTYYRSKWYNDYAVSVKSRITINPDTSKNQFSLQLNSVTPEDTAVYYCARDGDGGSYYDYYYYGMDVWGQGTTVTVSGGGGSGGGGSGGGGSDIQLTQSPSSLSTSVGDRVTITCRASQSISTYLNWYQQKPGKAPKLLIYAASNLQSGVPSRFSGSGSGTDFTLTISSLQPEDFATYFCQQSYTTPITFGQGTRLEIKTTTPAPRPPTPAPTIASQPLSLRPEACRPAAGGAVHTRGLDFACDIYIWAPLAGTCGVLLLSLVITLYCKRGRKKLLYIFKQPFMRPVQTTQEEDGCSCRFPEEEEGGCELRVKFSRSADAPAYQQGQNQLYNELNLGRREEYDVLDKRRGRDPEMGGKPRRKNPQEGLYNELQKDKMAEAYSEIGMKGERRRGKGHDGLYQGLSTATKDTYDALHMQALPPR

SEQ ID NO: 53 - protein, 484 aa, artificial sequence
  CAR 8 12
MALPVTALLLPLALLLHAARPQVQLQQSGPGLVKPSQTLSLTCAISGDSVSSNSAAWNWIRQSPSRGLEWLGRTYYRSAWYNDYAVSVKSRITINPDTSKNQFSLQLSSVTPEDTAVYYCARDVEGFDYWGQGTLVTVSGGGGSGGGGSGGGGSDIVMTQTPSSLSASVGDRVTITCRASQSISSYLNWYQQKPGKAPKLLIYAASSLQSGVPSRFSGSGSGTDFTLTISSLQPEDFATYYCQQSYSTPITFGQGTRLEIKTTTPAPRPPTPAPTIASQPLSLRPEACRPAAGGAVHTRGLDFACDIYIWAPLAGTCGVLLLSLVITLYCKRGRKKLLYIFKQPFMRPVQTTQEEDGCSCRFPEEEEGGCELRVKFSRSADAPAYQQGQNQLYNELNLGRREEYDVLDKRRGRDPEMGGKPRRKNPQEGLYNELQKDKMAEAYSEIGMKGERRRGKGHDGLYQGLSTATKDTYDALHMQALPPR

SEQ ID NO: 54 - protein, 489 aa, artificial sequence
  CAR 9 13
MALPVTALLLPLALLLHAARPQVQLQQSGPGLVKPSQTLSLTCAISGDSVSGNRATWNWIRQSPSRGLEWLGRTYYRSAWYNDYAVSVKGRITFNPDTSKNQFSLQLNSVTPEDTAVYYCARGESGAAADAFDIWGQGTTVTVSGGGGSGGGGSGGGGSDIQLTQSPPSLSASVGDRVTITCRASQSISSYLNWYQQKPGKAPKLLIYAASSLQSGVPSRFSGSGFGTDFTLTISSLQPEDFATYYCQQSYSTPQTFGQGTKVDIKTTTPAPRPPTPAPTIASQPLSLRPEACRPAAGGAVHTRGLDFACDIYIWAPLAGTCGVLLLSLVITLYCKRGRKKLLYIFKQPFMRPVQTTQEEDGCSCRFPEEEEGGCELRVKFSRSADAPAYQQGQNQLYNELNLGRREEYDVLDKRRGRDPEMGGKPRRKNPQEGLYNELQKDKMAEAYSEIGMKGERRRGKGHDGLYQGLSTATKDTYDALHMQALPPR

SEQ ID NO: 55 - protein, 489 aa, artificial sequence
  CAR 10 15
MALPVTALLLPLALLLHAARPQVQLVQSGAEVKKPGASVKVSCKASGYTFTSYYMHWVRQAPGQGLEWMGIINPSGGSTSYAQKFQGRVTMTRDTSTSTVYMELSSLRSEDTAVYYCAREDSGSGAFDIWGQGTLVTVSGGGGSGGGGSGGGGSEIVLTQSPLSLPVTPGEPASISCRSSRSLLSYHGYNYLDWYLQKPGQSPQLLIFVGSNRAPGVPDRFSGSGSGTDFTLNISRVEAEDVGVYYCMQSLQTPRTFGQGTKVEIKTTTPAPRPPTPAPTIASQPLSLRPEACRPAAGGAVHTRGLDFACDIYIWAPLAGTCGVLLLSLVITLYCKRGRKKLLYIFKQPFMRPVQTTQEEDGCSCRFPEEEEGGCELRVKFSRSADAPAYQQGQNQLYNELNLGRREEYDVLDKRRGRDPEMGGKPRRKNPQEGLYNELQKDKMAEAYSEIGMKGERRRGKGHDGLYQGLSTATKDTYDALHMQALPPR

SEQ ID NO: 56 - protein, 567 aa, artificial sequence
  1RQR3
MALPVTALLLPLALLLHAARPGGGGSCPYSNPSLCSGGGGSGGGGSQVQLQQSGPGLVKPSQTLSLTCAISGDSVSSNSAAWNWIRQSPSRGLEWLGRTYYRSTWYNDYAVSVKSRITINPDTSKNQFSLQLNSVTPEDTAVYYCAREVSGTSAFDIWGQGTMVTVSGGGGSGGGGSGGGGSDIQMTQSPSSLSASVGDRVTITCRASQSISSYLNWYQQKPGKAPKLLIYAASSLQSGVPSRFSGSGSGTDFTLTISSLQPEDFATYYCQQSYSTPLTFGGGTKLEIKGSGGGGSCPYSNPSLCSGGGGSELPTQGTFSNVSTNVSPAKPTTTACPYSNPSLCTTTPAPRPPTPAPTIASQPLSLRPEACRPAAGGAVHTRGLDFACDIYIWAPLAGTCGVLLLSLVITLYCKRGRKKLLYIFKQPFMRPVQTTQEEDGCSCRFPEEEEGGCELRVKFSRSADAPAYQQGQNQLYNELNLGRREEYDVLDKRRGRDPEMGGKPRRKNPQEGLYNELQKDKMAEAYSEIGMKGERRRGKGHDGLYQGLSTATKDTYDALHMQALPPR

SEQ ID NO: 57 - protein, 572 aa, artificial sequence
  2RQR3
MALPVTALLLPLALLLHAARPGGGGSCPYSNPSLCSGGGGSGGGGSQVQLQQSGPGLVKPSQTLSLTCAISGDSVSSNSAAWNWIRQSPSRGLEWLGRTYYRSKWYNDYAVSVKSRITINPDTSKNQFSLQLNSVTPEDTAVYYCARASMTGGYSYGDAFDIWGQGTLVTVSGGGGSGGGGSGGGGSAIRMTQSPSSLSASVGDRVTITCRASQSISSYLNWYQQKPGKAPKLLIYAASSLQSGVPSRFSGSGSGTDFSLTISSLQPEDSATYYCQQTYSTPLTFGQGTKVEIKGSGGGGSCPYSNPSLCSGGGGSELPTQGTFSNVSTNVSPAKPTTTACPYSNPSLCTTTPAPRPPTPAPTIASQPLSLRPEACRPAAGGAVHTRGLDFACDIYIWAPLAGTCGVLLLSLVITLYCKRGRKKLLYIFKQPFMRPVQTTQEEDGCSCRFPEEEEGGCELRVKFSRSADAPAYQQGQNQLYNELNLGRREEYDVLDKRRGRDPEMGGKPRRKNPQEGLYNELQKDKMAEAYSEIGMKGERRRGKGHDGLYQGLSTATKDTYDALHMQALPPR

SEQ ID NO: 58 - protein, 568 aa, artificial sequence
  3RQR3
MALPVTALLLPLALLLHAARPGGGGSCPYSNPSLCSGGGGSGGGGSQVQLQQSGPGLVEPSQTLSLTCAISGDSVSSDSVAWNWIRQSPSRGLEWLGRTYYRSTWYNDYAGSVKSRITINPDTSKNQFSLQLTSVTPEDTAVYYCTRSRHNTFRGMDVWGQGTTVTVSGGGGSGGGGSGGGGSDIVMTQSPSSLSASVGDRVTITCRASQTISSYLNWYQQKPGKAPKLLIYDASSLQSGVPSRFSGSGSGTDFTLTINSLQPEDFATYYCQQSYTTPITFGQGTRLEIKGSGGGGSCPYSNPSLCSGGGGSELPTQGTFSNVSTNVSPAKPTTTACPYSNPSLCTTTPAPRPPTPAPTIASQPLSLRPEACRPAAGGAVHTRGLDFACDIYIWAPLAGTCGVLLLSLVITLYCKRGRKKLLYIFKQPFMRPVQTTQEEDGCSCRFPEEEEGGCELRVKFSRSADAPAYQQGQNQLYNELNLGRREEYDVLDKRRGRDPEMGGKPRRKNPQEGLYNELQKDKMAEAYSEIGMKGERRRGKGHDGLYQGLSTATKDTYDALHMQALPPR

SEQ ID NO: 59 - protein, 568 aa, artificial sequence
  4RQR3
MALPVTALLLPLALLLHAARPGGGGSCPYSNPSLCSGGGGSGGGGSQVQLQQSGPGLVEPSQTLSLTCAISGDSVSSNSAAWNWIRQSPSRGLEWLGRTYYRSTWYNDYAGSVKSRITINPDTSKNQFSLQLTSVTPEDTAVYYCTRSRHNTFRGMDVWGQGTLVTVSGGGGSGGGGSGGGGSDIQLTQSPSSLSASVGDRVTITCRASQSISSYLNWYQQKPGKAPKLLIYAASSLQSGVPSRFSGSGSGTDFTLTISSLQPEDFATYYCQQSYSTPLTFGGGTKVEIKGSGGGGSCPYSNPSLCSGGGGSELPTQGTFSNVSTNVSPAKPTTTACPYSNPSLCTTTPAPRPPTPAPTIASQPLSLRPEACRPAAGGAVHTRGLDFACDIYIWAPLAGTCGVLLLSLVITLYCKRGRKKLLYIFKQPFMRPVQTTQEEDGCSCRFPEEEEGGCELRVKFSRSADAPAYQQGQNQLYNELNLGRREEYDVLDKRRGRDPEMGGKPRRKNPQEGLYNELQKDKMAEAYSEIGMKGERRRGKGHDGLYQGLSTATKDTYDALHMQALPPR

SEQ ID NO: 60 - protein, 564 aa, artificial sequence
  5RQR3
MALPVTALLLPLALLLHAARPGGGGSCPYSNPSLCSGGGGSGGGGSQVQLQQSGPGLVEPSQTLSLTCAISGDSVSSDSVAWNWIRQSPSRGLEWLGRTYYRSTWYNDYAGSVKSRITINPDTSKNQFSLQLNSVTPEDTAVYYCARDRNGMDVWGQGTMVTVSGGGGSGGGGSGGGGSDIVMTQSPSSLSASVGDRVTITCRASQSISSYLNWYQQKPGKAPKLLIYDASNLETGVPSRFSGSGSGTDFTFTITSLQPEDFATYYCQQSYTTPLTFGGGTKVEIKGSGGGGSCPYSNPSLCSGGGGSELPTQGTFSNVSTNVSPAKPTTTACPYSNPSLCTTTPAPRPPTPAPTIASQPLSLRPEACRPAAGGAVHTRGLDFACDIYIWAPLAGTCGVLLLSLVITLYCKRGRKKLLYIFKQPFMRPVQTTQEEDGCSCRFPEEEEGGCELRVKFSRSADAPAYQQGQNQLYNELNLGRREEYDVLDKRRGRDPEMGGKPRRKNPQEGLYNELQKDKMAEAYSEIGMKGERRRGKGHDGLYQGLSTATKDTYDALHMQALPPR

SEQ ID NO: 61 - protein, 567 aa, artificial sequence
  6RQR3
MALPVTALLLPLALLLHAARPGGGGSCPYSNPSLCSGGGGSGGGGSQVQLQQSGPGLVKPSQTLSLTCAISGDSVSSSSAAWNWIRQSPSRGLEWLGRTYYRSAWYNDYAVSVKSRITINPDTSKNQFSLQLNSVTPEDTAVYYCARESVLLDGMDVWGRGTTVTVSGGGGSGGGGSGGGGSAIRMTQSPSTLSASVGDRVTITCRASQSISTYLNWYQQKAGKAPRLLIHDASSLQSGVPSRFSGSGSGTDFTLTISSLQPEDFATYYCQQSYSTPLTFGGGTKVEIKGSGGGGSCPYSNPSLCSGGGGSELPTQGTFSNVSTNVSPAKPTTTACPYSNPSLCTTTPAPRPPTPAPTIASQPLSLRPEACRPAAGGAVHTRGLDFACDIYIWAPLAGTCGVLLLSLVITLYCKRGRKKLLYIFKQPFMRPVQTTQEEDGCSCRFPEEEEGGCELRVKFSRSADAPAYQQGQNQLYNELNLGRREEYDVLDKRRGRDPEMGGKPRRKNPQEGLYNELQKDKMAEAYSEIGMKGERRRGKGHDGLYQGLSTATKDTYDALHMQALPPR

SEQ ID NO: 62 - protein, 574 aa, artificial sequence
  7RQR3
MALPVTALLLPLALLLHAARPGGGGSCPYSNPSLCSGGGGSGGGGSQVQLQQSGPGLVQPSQTLSLTCVISGDSVSSNSATWNWIRQSPSRGLEWLGRTYYRSKWYNDYAVSVKSRITINPDTSKNQFSLQLNSVTPEDTAVYYCARDGDGGSYYDYYYYGMDVWGQGTTVTVSGGGGSGGGGSGGGGSDIQLTQSPSSLSTSVGDRVTITCRASQSISTYLNWYQQKPGKAPKLLIYAASNLQSGVPSRFSGSGSGTDFTLTISSLQPEDFATYFCQQSYTTPITFGQGTRLEIKGSGGGGSCPYSNPSLCSGGGGSELPTQGTFSNVSTNVSPAKPTTTACPYSNPSLCTTTPAPRPPTPAPTIASQPLSLRPEACRPAAGGAVHTRGLDFACDIYIWAPLAGTCGVLLLSLVITLYCKRGRKKLLYIFKQPFMRPVQTTQEEDGCSCRFPEEEEGGCELRVKFSRSADAPAYQQGQNQLYNELNLGRREEYDVLDKRRGRDPEMGGKPRRKNPQEGLYNELQKDKMAEAYSEIGMKGERRRGKGHDGLYQGLSTATKDTYDALHMQALPPR

SEQ ID NO: 63 - protein, 564 aa, artificial sequence
  8RQR3
MALPVTALLLPLALLLHAARPGGGGSCPYSNPSLCSGGGGSGGGGSQVQLQQSGPGLVKPSQTLSLTCAISGDSVSSNSAAWNWIRQSPSRGLEWLGRTYYRSAWYNDYAVSVKSRITINPDTSKNQFSLQLSSVTPEDTAVYYCARDVEGFDYWGQGTLVTVSGGGGSGGGGSGGGGSDIVMTQTPSSLSASVGDRVTITCRASQSISSYLNWYQQKPGKAPKLLIYAASSLQSGVPSRFSGSGSGTDFTLTISSLQPEDFATYYCQQSYSTPITFGQGTRLEIKGSGGGGSCPYSNPSLCSGGGGSELPTQGTFSNVSTNVSPAKPTTTACPYSNPSLCTTTPAPRPPTPAPTIASQPLSLRPEACRPAAGGAVHTRGLDFACDIYIWAPLAGTCGVLLLSLVITLYCKRGRKKLLYIFKQPFMRPVQTTQEEDGCSCRFPEEEEGGCELRVKFSRSADAPAYQQGQNQLYNELNLGRREEYDVLDKRRGRDPEMGGKPRRKNPQEGLYNELQKDKMAEAYSEIGMKGERRRGKGHDGLYQGLSTATKDTYDALHMQALPPR

SEQ ID NO: 64 - protein, 569 aa, artificial sequence
  9RQR3
MALPVTALLLPLALLLHAARPGGGGSCPYSNPSLCSGGGGSGGGGSQVQLQQSGPGLVKPSQTLSLTCAISGDSVSGNRATWNWIRQSPSRGLEWLGRTYYRSAWYNDYAVSVKGRITFNPDTSKNQFSLQLNSVTPEDTAVYYCARGESGAAADAFDIWGQGTTVTVSGGGGSGGGGSGGGGSDIQLTQSPPSLSASVGDRVTITCRASQSISSYLNWYQQKPGKAPKLLIYAASSLQSGVPSRFSGSGFGTDFTLTISSLQPEDFATYYCQQSYSTPQTFGQGTKVDIKGSGGGGSCPYSNPSLCSGGGGSELPTQGTFSNVSTNVSPAKPTTTACPYSNPSLCTTTPAPRPPTPAPTIASQPLSLRPEACRPAAGGAVHTRGLDFACDIYIWAPLAGTCGVLLLSLVITLYCKRGRKKLLYIFKQPFMRPVQTTQEEDGCSCRFPEEEEGGCELRVKFSRSADAPAYQQGQNQLYNELNLGRREEYDVLDKRRGRDPEMGGKPRRKNPQEGLYNELQKDKMAEAYSEIGMKGERRRGKGHDGLYQGLSTATKDTYDALHMQALPPR

SEQ ID NO: 65 - protein, 569 aa, artificial sequence
  10RQR3
MALPVTALLLPLALLLHAARPGGGGSCPYSNPSLCSGGGGSGGGGSQVQLVQSGAEVKKPGASVKVSCKASGYTFTSYYMHWVRQAPGQGLEWMGIINPSGGSTSYAQKFQGRVTMTRDTSTSTVYMELSSLRSEDTAVYYCAREDSGSGAFDIWGQGTLVTVSGGGGSGGGGSGGGGSEIVLTQSPLSLPVTPGEPASISCRSSRSLLSYHGYNYLDWYLQKPGQSPQLLIFVGSNRAPGVPDRFSGSGSGTDFTLNISRVEAEDVGVYYCMQSLQTPRTFGQGTKVEIKGSGGGGSCPYSNPSLCSGGGGSELPTQGTFSNVSTNVSPAKPTTTACPYSNPSLCTTTPAPRPPTPAPTIASQPLSLRPEACRPAAGGAVHTRGLDFACDIYIWAPLAGTCGVLLLSLVITLYCKRGRKKLLYIFKQPFMRPVQTTQEEDGCSCRFPEEEEGGCELRVKFSRSADAPAYQQGQNQLYNELNLGRREEYDVLDKRRGRDPEMGGKPRRKNPQEGLYNELQKDKMAEAYSEIGMKGERRRGKGHDGLYQGLSTATKDTYDALHMQALPPR

SEQ ID NO: 66 - protein, 528 aa, artificial sequence
  CAR4 R2
MALPVTALLLPLALLLHAARPQVQLQQSGPGLVEPSQTLSLTCAISGDSVSSNSAAWNWIRQSPSRGLEWLGRTYYRSTWYNDYAGSVKSRITINPDTSKNQFSLQLTSVTPEDTAVYYCTRSRHNTFRGMDVWGQGTLVTVSGGGGSGGGGSGGGGSDIQLTQSPSSLSASVGDRVTITCRASQSISSYLNWYQQKPGKAPKLLIYAASSLQSGVPSRFSGSGSGTDFTLTISSLQPEDFATYYCQQSYSTPLTFGGGTKVEIKSDPGSGGGGSCPYSNPSLCSGGGGSCPYSNPSLCSGGGGSTTTPAPRPPTPAPTIASQPLSLRPEACRPAAGGAVHTRGLDFACDIYIWAPLAGTCGVLLLSLVITLYCKRGRKKLLYIFKQPFMRPVQTTQEEDGCSCRFPEEEEGGCELRVKFSRSADAPAYQQGQNQLYNELNLGRREEYDVLDKRRGRDPEMGGKPRRKNPQEGLYNELQKDKMAEAYSEIGMKGERRRGKGHDGLYQGLSTATKDTYDALHMQALPPR

SEQ ID NO: 67 - protein, 534 aa, artificial sequence
  CAR7R2
MALPVTALLLPLALLLHAARPQVQLQQSGPGLVQPSQTLSLTCVISGDSVSSNSATWNWIRQSPSRGLEWLGRTYYRSKWYNDYAVSVKSRITINPDTSKNQFSLQLNSVTPEDTAVYYCARDGDGGSYYDYYYYGMDVWGQGTTVTVSGGGGSGGGGSGGGGSDIQLTQSPSSLSTSVGDRVTITCRASQSISTYLNWYQQKPGKAPKLLIYAASNLQSGVPSRFSGSGSGTDFTLTISSLQPEDFATYFCQQSYTTPITFGQGTRLEIKSDPGSGGGGSCPYSNPSLCSGGGGSCPYSNPSLCSGGGGSTTTPAPRPPTPAPTIASQPLSLRPEACRPAAGGAVHTRGLDFACDIYIWAPLAGTCGVLLLSLVITLYCKRGRKKLLYIFKQPFMRPVQTTQEEDGCSCRFPEEEEGGCELRVKFSRSADAPAYQQGQNQLYNELNLGRREEYDVLDKRRGRDPEMGGKPRRKNPQEGLYNELQKDKMAEAYSEIGMKGERRRGKGHDGLYQGLSTATKDTYDALHMQALPPR

SEQ ID NO: 68 - protein, 529 aa, artificial sequence
  CAR9R2
MALPVTALLLPLALLLHAARPQVQLQQSGPGLVKPSQTLSLTCAISGDSVSGNRATWNWIRQSPSRGLEWLGRTYYRSAWYNDYAVSVKGRITFNPDTSKNQFSLQLNSVTPEDTAVYYCARGESGAAADAFDIWGQGTTVTVSGGGGSGGGGSGGGGSDIQLTQSPPSLSASVGDRVTITCRASQSISSYLNWYQQKPGKAPKLLIYAASSLQSGVPSRFSGSGFGTDFTLTISSLQPEDFATYYCQQSYSTPQTFGQGTKVDIKSDPGSGGGGSCPYSNPSLCSGGGGSCPYSNPSLCSGGGGSTTTPAPRPPTPAPTIASQPLSLRPEACRPAAGGAVHTRGLDFACDIYIWAPLAGTCGVLLLSLVITLYCKRGRKKLLYIFKQPFMRPVQTTQEEDGCSCRFPEEEEGGCELRVKFSRSADAPAYQQGQNQLYNELNLGRREEYDVLDKRRGRDPEMGGKPRRKNPQEGLYNELQKDKMAEAYSEIGMKGERRRGKGHDGLYQGLSTATKDTYDALHMQALPPR

SEQ ID NO: 69 - protein, 529 aa, artificial sequence
  CAR10R2
MALPVTALLLPLALLLHAARPQVQLVQSGAEVKKPGASVKVSCKASGYTFTSYYMHWVRQAPGQGLEWMGIINPSGGSTSYAQKFQGRVTMTRDTSTSTVYMELSSLRSEDTAVYYCAREDSGSGAFDIWGQGTLVTVSGGGGSGGGGSGGGGSEIVLTQSPLSLPVTPGEPASISCRSSRSLLSYHGYNYLDWYLQKPGQSPQLLIFVGSNRAPGVPDRFSGSGSGTDFTLNISRVEAEDVGVYYCMQSLQTPRTFGQGTKVEIKSDPGSGGGGSCPYSNPSLCSGGGGSCPYSNPSLCSGGGGSTTTPAPRPPTPAPTIASQPLSLRPEACRPAAGGAVHTRGLDFACDIYIWAPLAGTCGVLLLSLVITLYCKRGRKKLLYIFKQPFMRPVQTTQEEDGCSCRFPEEEEGGCELRVKFSRSADAPAYQQGQNQLYNELNLGRREEYDVLDKRRGRDPEMGGKPRRKNPQEGLYNELQKDKMAEAYSEIGMKGERRRGKGHDGLYQGLSTATKDTYDALHMQALPPR

SEQ ID NO: 70 - DNA, 59 bp, artificial sequence
  TARGET TALEN(R)
  misc_feature (44): r is a or g
rgatcctcttgtcccacagatatccagaaccctgaccctgccgrgtaccagctgagaga

SEQ ID NO: 71 - protein, 121 aa, artificial sequence
  VH CAR1
QVQLQQSGPGLVKPSQTLSLTCAISGDSVSSNSAAWNWIRQSPSRGLEWLGRTYYRSTWYNDYAVSVKSRITINPDTSKNQFSLQLNSVTPEDTAVYYCAREVSGTSAFDIWGQGTMVTVS

SEQ ID NO: 72 - protein, 107 aa, artificial sequence
  VL CAR1
DIQMTQSPSSLSASVGDRVTITCRASQSISSYLNWYQQKPGKAPKLLIYAASSLQSGVPSRFSGSGSGTDFTLTISSLQPEDFATYYCQQSYSTPLTFGGGTKLEIK

SEQ ID NO: 73 - protein, 126 aa, artificial sequence
  VH CAR2
QVQLQQSGPGLVKPSQTLSLTCAISGDSVSSNSAAWNWIRQSPSRGLEWLGRTYYRSKWYNDYAVSVKSRITINPDTSKNQFSLQLNSVTPEDTAVYYCARASMTGGYSYGDAFDIWGQGTLVTVS

SEQ ID NO: 74 - protein, 107 aa, artificial sequence
  VL CAR2
AIRMTQSPSSLSASVGDRVTITCRASQSISSYLNWYQQKPGKAPKLLIYAASSLQSGVPSRFSGSGSGTDFSLTISSLQPEDSATYYCQQTYSTPLTFGQGTKVEIK

SEQ ID NO: 75 - protein, 122 aa, artificial sequence
  VH CAR3
QVQLQQSGPGLVEPSQTLSLTCAISGDSVSSDSVAWNWIRQSPSRGLEWLGRTYYRSTWYNDYAGSVKSRITINPDTSKNQFSLQLTSVTPEDTAVYYCTRSRHNTFRGMDVWGQGTTVTVS

SEQ ID NO: 76 - protein, 107 aa, artificial sequence
  VL CAR3
DIVMTQSPSSLSASVGDRVTITCRASQTISSYLNWYQQKPGKAPKLLIYDASSLQSGVPSRFSGSGSGTDFTLTINSLQPEDFATYYCQQSYTTPITFGQGTRLEIK

SEQ ID NO: 77 - protein, 122 aa, artificial sequence
  VH CAR4
QVQLQQSGPGLVEPSQTLSLTCAISGDSVSSNSAAWNWIRQSPSRGLEWLGRTYYRSTWYNDYAGSVKSRITINPDTSKNQFSLQLTSVTPEDTAVYYCTRSRHNTFRGMDVWGQGTLVTVS

SEQ ID NO: 78 - protein, 107 aa, artificial sequence
  VL CAR4
DIQLTQSPSSLSASVGDRVTITCRASQSISSYLNWYQQKPGKAPKLLIYAASSLQSGVPSRFSGSGSGTDFTLTISSLQPEDFATYYCQQSYSTPLTFGGGTKVEIK

SEQ ID NO: 79 - protein, 118 aa, artificial sequence
  VH CAR5
QVQLQQSGPGLVEPSQTLSLTCAISGDSVSSDSVAWNWIRQSPSRGLEWLGRTYYRSTWYNDYAGSVKSRITINPDTSKNQFSLQLNSVTPEDTAVYYCARDRNGMDVWGQGTMVTVS

SEQ ID NO: 80 - protein, 107 aa, artificial sequence
  VL CAR5
DIVMTQSPSSLSASVGDRVTITCRASQSISSYLNWYQQKPGKAPKLLIYDASNLETGVPSRFSGSGSGTDFTFTITSLQPEDFATYYCQQSYTTPLTFGGGTKVEIK

SEQ ID NO: 81 - protein, 121 aa, artificial sequence
  VH CAR6
QVQLQQSGPGLVKPSQTLSLTCAISGDSVSSSSAAWNWIRQSPSRGLEWLGRTYYRSAWYNDYAVSVKSRITINPDTSKNQFSLQLNSVTPEDTAVYYCARESVLLDGMDVWGRGTTVTVS

SEQ ID NO: 82 - protein, 107 aa, artificial sequence
  VL CAR6
AIRMTQSPSTLSASVGDRVTITCRASQSISTYLNWYQQKAGKAPRLLIHDASSLQSGVPSRFSGSGSGTDFTLTISSLQPEDFATYYCQQSYSTPLTFGGGTKVEIK

SEQ ID NO: 83 - protein, 128 aa, artificial sequence
  VH CAR7
QVQLQQSGPGLVQPSQTLSLTCVISGDSVSSNSATWNWIRQSPSRGLEWLGRTYYRSKWYNDYAVSVKSRITINPDTSKNQFSLQLNSVTPEDTAVYYCARDGDGGSYYDYYYYGMDVWGQGTTVTVS

SEQ ID NO: 84 - protein, 107 aa, artificial sequence
  VL CAR7
DIQLTQSPSSLSTSVGDRVTITCRASQSISTYLNWYQQKPGKAPKLLIYAASNLQSGVPSRFSGSGSGTDFTLTISSLQPEDFATYFCQQSYTTPITFGQGTRLEIK

SEQ ID NO: 85 - protein, 118 aa, artificial sequence
  VH CAR8
QVQLQQSGPGLVKPSQTLSLTCAISGDSVSSNSAAWNWIRQSPSRGLEWLGRTYYRSAWYNDYAVSVKSRITINPDTSKNQFSLQLSSVTPEDTAVYYCARDVEGFDYWGQGTLVTVS

SEQ ID NO: 86 - protein, 107 aa, artificial sequence
  VL CAR8
DIVMTQTPSSLSASVGDRVTITCRASQSISSYLNWYQQKPGKAPKLLIYAASSLQSGVPSRFSGSGSGTDFTLTISSLQPEDFATYYCQQSYSTPITFGQGTRLEIK

SEQ ID NO: 87 - protein, 123 aa, artificial sequence
  VH CAR9
QVQLQQSGPGLVKPSQTLSLTCAISGDSVSGNRATWNWIRQSPSRGLEWLGRTYYRSAWYNDYAVSVKGRITFNPDTSKNQFSLQLNSVTPEDTAVYYCARGESGAAADAFDIWGQGTTVTVS

SEQ ID NO: 88 - protein, 107 aa, artificial sequence
  VL CAR9
DIQLTQSPPSLSASVGDRVTITCRASQSISSYLNWYQQKPGKAPKLLIYAASSLQSGVPSRFSGSGFGTDFTLTISSLQPEDFATYYCQQSYSTPQTFGQGTKVDIK

SEQ ID NO: 89 - protein, 118 aa, artificial sequence
  VH CAR10
QVQLVQSGAEVKKPGASVKVSCKASGYTFTSYYMHWVRQAPGQGLEWMGIINPSGGSTSYAQKFQGRVTMTRDTSTSTVYMELSSLRSEDTAVYYCAREDSGSGAFDIWGQGTLVTVS

SEQ ID NO: 90 - protein, 112 aa, artificial sequence
  VL CAR10
EIVLTQSPLSLPVTPGEPASISCRSSRSLLSYHGYNYLDWYLQKPGQSPQLLIFVGSNRAPGVPDRFSGSGSGTDFTLNISRVEAEDVGVYYCMQSLQTPRTFGQGTKVEIK

SEQ ID NO: 91 - protein, 9 aa, artificial sequence
  R
CPYSNPSLC

SEQ ID NO: 92 - protein, 24 aa, artificial sequence
  Q
ELPTQGTFSNVSTNVSPAKPTTTA

SEQ ID NO: 93 - protein, 489 aa, artificial sequence
  CAR distal CD22
MALPVTALLLPLALLLHAARPEVQLVESGGGLVKPGGSLKLSCAASGFAFSIYDMSWVRQTPEKRLEWVAYISSGGGTYYPDTVKGRFTISRDNAKNTLYLQMSSLKSEDTAMYYCARHSGYGTHWGVLFAYWGQGTLVTVSAGGGGSGGGGSGGGGSDIQMTQTTSSLSASLGDRVTISCRASQDISNYLNWYQQKPDGTVKLLIYYTSILHSGVPSRFSGSGSGTDYSLTISNLEQEDFATYFCQQGNTLPWTFGGGTKLEIKATTTPAPRPPTPAPTIASQPLSLRPEACRPAAGGAVHTRGLDFACDIYIWAPLAGTCGVLLLSLVITLYCKRGRKKLLYIFKQPFMRPVQTTQEEDGCSCRFPEEEEGGCELRVKFSRSADAPAYQQGQNQLYNELNLGRREEYDVLDKRRGRDPEMGGKPRRKNPQEGLYNELQKDKMAEAYSEIGMKGERRRGKGHDGLYQGLSTATKDTYDALHMQALPPR

SEQ ID NO: 94 - DNA, 1470 bp, artificial sequence
  CAR distal CD22
atggctctgcccgtcaccgctctgctgctgccactggccctgctgctgcacgcagcaaggcctgaggtgcagctggtggaatccggaggaggcctggtgaagcctggcggctctctgaagctgagctgtgccgcctccggcttcgccttttccatctacgacatgtcttgggtgaggcagaccccagagaagcgcctggagtgggtggcctatatcagctccggcggcggcacctactatcccgacacagtgaagggccggttcaccatctctagagataacgccaagaatacactgtacctgcagatgtctagcctgaagagcgaggataccgccatgtactattgcgcaaggcactccggatacggaacacactggggcgtgctgtttgcctattggggccagggcaccctggtgacagtgagcgccggaggaggaggaagcggcggaggaggctccggcggcggcggctctgacatccagatgacccagaccacatcctctctgagcgcctccctgggcgacagggtgacaatctcttgtagagccagccaggatatctccaactacctgaattggtatcagcagaagcctgatggcaccgtgaagctgctgatctactatacatctatcctgcacagcggagtgccatcccggttctctggaagcggatccggaaccgactactctctgacaatcagcaacctggagcaggaggatttcgccacctatttttgccagcagggcaataccctgccttggacatttggcggcggcacaaagctggagatcaaggccaccacaacccctgcaccaaggccaccaacaccagcacctaccatcgcatctcagcctctgagcctgagaccagaggcatgtaggccagcagcaggaggagcagtgcacacaaggggactggattttgcctgtgatatctacatctgggcacctctggcaggaacatgtggcgtgctcctgctcagcctggtcatcaccctgtactgcaagagaggcaggaagaagctgctgtatatcttcaagcagcccttcatgagacccgtgcagacaacccaggaggaggacggctgctcctgtaggttcccagaagaggaggagggaggatgtgagctgcgcgtgaagttttcccggtctgccgatgcacctgcataccagcagggacagaatcagctgtataacgagctgaatctgggccggagagaggagtacgacgtgctggataagaggaggggaagggacccagagatgggaggcaagcctcggagaaagaacccacaggagggcctgtacaatgagctgcagaaggacaagatggccgaggcctattctgagatcggcatgaagggagagaggcgccggggcaagggacacgatggcctgtaccagggcctgtccacagccaccaaggacacctatgatgccctgcatatgcaggcactgcctccaaggtga

SEQ ID NO: 95 - protein, 495 aa, artificial sequence
  description of artificial sequence: synthetic polypeptide
  4G7-CAR version 1
MALPVTALLLPLALLLHAARPEVQLQQSGPELIKPGASVKMSCKASGYTFTSYVMHWVKQKPGQGLEWIGYINPYNDGTKYNEKFKGKATLTSDKSSSTAYMELSSLTSEDSAVYYCARGTYYYGSRVFDYWGQGTTLTVSSGGGGSGGGGSGGGGSDIVMTQAAPSIPVTPGESVSISCRSSKSLLNSNGNTYLYWFLQRPGQSPQLLIYRMSNLASGVPDRFSGSGSGTAFTLRISRVEAEDVGVYYCMQHLEYPFTFGAGTKLELKRADTTTPAPRPPTPAPTIASQPLSLRPEACRPAAGGAVHTRGLDFACDIYIWAPLAGTCGVLLLSLVITLYCKRGRKKLLYIFKQPFMRPVQTTQEEDGCSCRFPEEEEGGCELRVKFSRSADAPAYQQGQNQLYNELNLGRREEYDVLDKRRGRDPEMGGKPRRKNPQEGLYNELQKDKMAEAYSEIGMKGERRRGKGHDGLYQGLSTATKDTYDALHMQALPPR

SEQ ID NO: 96 - protein, 495 aa, artificial sequence
  description of artificial sequence: synthetic polypeptide
  4G7-CAR version 2
METDTLLLWVLLLWVPGSTGEVQLQQSGPELIKPGASVKMSCKASGYTFTSYVMHWVKQKPGQGLEWIGYINPYNDGTKYNEKFKGKATLTSDKSSSTAYMELSSLTSEDSAVYYCARGTYYYGSRVFDYWGQGTTLTVSSGGGGSGGGGSGGGGSDIVMTQAAPSIPVTPGESVSISCRSSKSLLNSNGNTYLYWFLQRPGQSPQLLIYRMSNLASGVPDRFSGSGSGTAFTLRISRVEAEDVGVYYCMQHLEYPFTFGAGTKLELKRSDPTTTPAPRPPTPAPTIASQPLSLRPEACRPAAGGAVHTRGLDFACDIYIWAPLAGTCGVLLLSLVITLYCKRGRKKLLYIFKQPFMRPVQTTQEEDGCSCRFPEEEEGGCELRVKFSRSADAPAYQQGQNQLYNELNLGRREEYDVLDKRRGRDPEMGGKPRRKNPQEGLYNELQKDKMAEAYSEIGMKGERRRGKGHDGLYQGLSTATKDTYDALHMQALPPR

SEQ ID NO: 97 - protein, 5 aa, Artificial Sequence
  pentapeptide linker
GGGGS

SEQ ID NO: 98 - protein, 18 aa, Artificial Sequence
  18-mer linker
GGSSRSSSSGGGGSGGGG

SEQ ID NO: 99 - protein, 15 aa, Artificial Sequence
  15-mer linker
RGRGRGRGRSRGGGS

SEQ ID NO: 100 - protein, 4 aa, Artificial Sequence
  Linker
GGGS

SEQ ID NO: 101 - protein, 4 aa, Artificial Sequence
  Linker
SGGS

SEQ ID NO: 102 - protein, 5 aa, Artificial Sequence
  Linker
SSGGS

SEQ ID NO: 103 - protein, 4 aa, Artificial Sequence
  Linker
GGGG

SEQ ID NO: 104 - protein, 5 aa, Artificial Sequence
  Linker
SGGGG

SEQ ID NO: 105 - protein, 6 aa, Artificial Sequence
  Linker
SGGGGS

SEQ ID NO: 106 - protein, 6 aa, Artificial Sequence
  Linker
GGGGGS

SEQ ID NO: 107 - protein, 7 aa, Artificial Sequence
  Linker
SGGGGGS

SEQ ID NO: 108 - protein, 6 aa, Artificial Sequence
  Linker
SGGGGG

SEQ ID NO: 109 - protein, 7 aa, Artificial Sequence
  Linker
GSGGGGS

SEQ ID NO: 110 - protein, 8 aa, Artificial Sequence
  Linker
GGGGGGGS

SEQ ID NO: 111 - protein, 8 aa, Artificial Sequence
  Linker
SGGGGGGG

SEQ ID NO: 112 - protein, 9 aa, Artificial Sequence
  Linker
SGGGGGGGS

SEQ ID NO: 113 - protein, 11 aa, Artificial Sequence
  Linker
SGGGGSGGGGS

SEQ ID NO: 114 - protein, 24 aa, Artificial Sequence
  mAb-specific epitope
NSELLSLINDMPITNDQKKLMSNN

SEQ ID NO: 115 - protein, 12 aa, Artificial Sequence
  mAb-specific epitope
CQFDLSTRRLKC

SEQ ID NO: 116 - protein, 12 aa, Artificial Sequence
  mAb-specific epitope
CQYNLSSRALKC

SEQ ID NO: 117 - protein, 12 aa, Artificial Sequence
  mAb-specific epitope
CVWQRWQKSYVC

SEQ ID NO: 118 - protein, 12 aa, Artificial Sequence
  mAb-specific epitope
CMWDRFSRWYKC

SEQ ID NO: 119 - protein, 25 aa, Artificial Sequence
  mAb-specific epitope
SFVLNWYRMSPSNQTDKLAAFPEDR

SEQ ID NO: 120 - protein, 19 aa, Artificial Sequence
  mAb-specific epitope
SGTYLCGAISLAPKAQIKE

SEQ ID NO: 121 - protein, 12 aa, Artificial Sequence
  mAb-specific epitope
GQNDTSQTSSPS

SEQ ID NO: 122 - protein, 15 aa, Artificial Sequence
  Linker
GGGGSGGGGSGGGGS

SEQ ID NO: 123 - DNA, 16 bp, Artificial Sequence
  TRAC target sequence
ttgtcccacagatatc

SEQ ID NO: 124 - DNA, 19 bp, Artificial Sequence
  TRAC target sequence
ttgtcccacagatatccag

SEQ ID NO: 125 - DNA, 15 bp, Artificial Sequence
  Sequence cleaved by TALEN
agaaccctgaccctg

SEQ ID NO: 126 - DNA, 49 bp, Artificial Sequence
  Target sequence
ttgtcccacagatatccagaaccctgaccctgccgtgtaccagctgaga